European Patent Application EP 4 524 248 A1, published March 19, 2025. Title: anti-TAA-anti-CD3 multispecific antibody. Applicant: Astellas Pharma Inc. The sequence listing filed with the application follows.

SEQUENCE LISTING (67 sequences)

SEQ ID NO: 1 - DNA, 1353 bp, synthetic construct
  source 1..1353: mol_type = other DNA
  CDS 1..1353: protein_id = 2; translation = QVQLVESGGGVVQPGGSLRLSCAASGFTFSSYGMHWVRQAPGKGLEWVAVIWYDGRNKYYADSVKGRFTISRDNSKNTLYLQMNSLRAEDTAVYYCTRDHSGSGSYYIDYWGQGTLVTVSSASTKGPSVFPLAPSSKSTSGGTAALGCLVKDYFPEPVTVSWNSGALTSGVHTFPAVLQSSGLYSLSSVVTVPSSSLGTQTYICNVNHKPSNTKVDKKVEPKSCDKTHTCPPCPAPEAAGGPSVFLFPPKPKDTLMISRTPEVTCVVVDVSHEDPEVKFNWYVDGVEVHNAKTKPREEQYGSTYRVVSVLTVLHQDWLNGKEYKCKVSNKALPAPIEKTISKAKGQPREPQVYTLPPSRDELTKNQVSLSCAVKGFYPSDIAVEWESNGQPENNYKTTPPVLDSDGSFFLVSKLTVDKSRWQQGNVFSCSVMHEALHNHYTQKSLSLSPGK
caggttcagctggttgaatctggcggcggagttgttcagcctggcggatctctgagactgtcttgtgccgcctccggcttcaccttctcctcttacggaatgcactgggtccgacaggcccctggcaaaggattggaatgggtcgccgtgatttggtacgacggccggaacaagtactacgccgactccgtgaagggcagattcaccatctctcgggacaactccaagaacaccctgtacctgcagatgaactccctgagagccgaggacaccgccgtgtactactgcaccagagatcactccggctccggcagctactacatcgattattggggccagggcaccctggtcaccgtttcttccgctagcaccaagggacccagcgtgttccctctggctccttccagcaagtctacctctggcggaacagctgctctgggctgcctggtcaaggactactttcctgagcctgtgaccgtgtcctggaactctggcgctctgacatctggcgtgcacacctttccagctgtgctgcagtcctccggcctgtactctctgtcctctgtcgtgaccgtgccttccagctctctgggaacccagacctacatctgcaatgtgaaccacaagccttccaacaccaaggtggacaagaaggtggaacccaagtcctgcgacaagacccacacctgtcctccatgtcctgctccagaagctgctggcggcccttccgtgtttctgttccctccaaagcctaaggacaccctgatgatctctcggacccctgaagtgacctgcgtggtggtggatgtgtctcacgaggacccagaagtgaagttcaattggtacgtggacggcgtggaagtgcacaacgccaagaccaagcctagagaggaacagtacggctccacctacagagtggtgtccgtgctgacagtgctgcaccaggattggctgaacggcaaagagtacaagtgcaaggtgtccaacaaggccctgcctgctcctatcgaaaagaccatctccaaggccaagggccagcctagggaaccccaggtttacaccttgcctccatctcgggacgagctgaccaagaaccaggtgtccctgtcttgcgctgtgaagggcttctacccctccgatatcgccgtggaatgggagtctaatggccagcctgagaacaactacaagacaacccctcctgtgctggactccgacggctcattcttcctggtgtccaagctgaccgtggacaagtctagatggcagcagggcaacgtgttctcctgcagcgtgatgcacgaggccctgcacaatcactacacacagaagtctctgtctctgagccccggcaag

SEQ ID NO: 2 - protein, 451 aa, synthetic construct
QVQLVESGGGVVQPGGSLRLSCAASGFTFSSYGMHWVRQAPGKGLEWVAVIWYDGRNKYYADSVKGRFTISRDNSKNTLYLQMNSLRAEDTAVYYCTRDHSGSGSYYIDYWGQGTLVTVSSASTKGPSVFPLAPSSKSTSGGTAALGCLVKDYFPEPVTVSWNSGALTSGVHTFPAVLQSSGLYSLSSVVTVPSSSLGTQTYICNVNHKPSNTKVDKKVEPKSCDKTHTCPPCPAPEAAGGPSVFLFPPKPKDTLMISRTPEVTCVVVDVSHEDPEVKFNWYVDGVEVHNAKTKPREEQYGSTYRVVSVLTVLHQDWLNGKEYKCKVSNKALPAPIEKTISKAKGQPREPQVYTLPPSRDELTKNQVSLSCAVKGFYPSDIAVEWESNGQPENNYKTTPPVLDSDGSFFLVSKLTVDKSRWQQGNVFSCSVMHEALHNHYTQKSLSLSPGK

SEQ ID NO: 3 - DNA, 639 bp, synthetic construct
  CDS 1..639: protein_id = 4; translation = EIAMTQSPATLSVSPGERATLSCRASQSVSSNLAWYQQKPGQAPRLLIYGASTRATGLPARFSGSGSGTEFTLTISSLQSEDFAVYYCQQYNNFWTFGQGTKVEIKRTVAAPSVFIFPPSDEQLKSGTASVVCLLNNFYPREAKVQWKVDNALQSGNSQESVTEQDSKDSTYSLSSTLTLSKADYEKHKVYACEVTHQGLSSPVTKSFNRGEC
  source 1..639: mol_type = other DNA
gagattgccatgacacagtctcccgccacactgtctgttagccctggcgagagagctaccctgtcctgtagagcctctcagtccgtgtcctctaacctggcctggtatcagcagaagcctggacaggctccccggctgttgatctatggcgcttctaccagagctaccggcctgcctgctagattctccggctctggatctggcaccgagtttaccctgaccatctccagcctgcagtccgaggatttcgccgtgtactactgccagcagtacaacaacttctggaccttcggccagggcaccaaggtggaaatcaagcgtacggtggccgctccttccgtgttcatcttcccaccttccgacgagcagctgaagtccggcacagcttctgtcgtgtgcctgctgaacaacttttaccctcgggaagccaaggtgcagtggaaggtggacaatgccctgcagagcggcaactcccaagagtctgtgaccgagcaggactccaaggacagcacctacagcctgtcctccacactgaccctgtccaaggccgactacgagaagcacaaggtgtacgcctgcgaagtgacccatcagggcctgtctagccctgtgaccaagtctttcaaccggggcgagtgt

SEQ ID NO: 4 - protein, 213 aa, synthetic construct
EIAMTQSPATLSVSPGERATLSCRASQSVSSNLAWYQQKPGQAPRLLIYGASTRATGLPARFSGSGSGTEFTLTISSLQSEDFAVYYCQQYNNFWTFGQGTKVEIKRTVAAPSVFIFPPSDEQLKSGTASVVCLLNNFYPREAKVQWKVDNALQSGNSQESVTEQDSKDSTYSLSSTLTLSKADYEKHKVYACEVTHQGLSSPVTKSFNRGEC

SEQ ID NO: 5 - DNA, 1458 bp, synthetic construct
  CDS 1..1458: protein_id = 6; translation = EVQLVESGGGLIQPGGSLRLSCAASGFTFNTYAMNWVRQAPGKGLEWVARIRSKYNNYATYYADSVKDRFTISRDDSKSTLYLQMNNLRAEDTAVYYCVRHGNFGNSYVSWFAYWGQGTLVTVSSGKPGSGKPGSGKPGSGKPGSQAVVTQEPSLTVSPGGTVTLTCRSSTGAVTTSNYANWVQQKPGQAPRGLIGGTNKRAPGTPARFSGSLLGDKAALTLSGAQPEDEAEYYCALWYSNLWVFGGGTKVTVLEPKSSDKTHTCPPCPAPEAAGGPSVFLFPPKPKDTLMISRTPEVTCVVVDVSHEDPEVKFNWYVDGVEVHNAKTKPREEQYGSTYRVVSVLTVLHQDWLNGKEYKCKVSNKALPAPIEKTISKAKGQPREPQVYTLPPSRDELTKNQVSLWCLVKGFYPSDIAVEWESNGQPENNYKTTPPVLDSDGSFFLYSKLTVDKSRWQQGNVFSCSVMHEALHNHYTQKSLSLSPGK
  source 1..1458: mol_type = other DNA
gaagtgcagctggttgaatctggcggcggactgattcagcctggcggatctctgagactgtcttgtgccgcctctggcttcaccttcaacacctacgccatgaactgggtccgacaggctcctggcaaaggcctggaatgggtcgcccggatcagatccaagtacaacaattacgccacctactacgccgactccgtgaaggaccggttcaccatctctcgggacgactccaagagcaccctgtacctgcagatgaacaacctgagagccgaggacaccgccgtgtactactgtgtgcggcacggcaacttcggcaactcctatgtgtcttggtttgcctactggggccagggcacactggtcacagtgtcctctggaaagcctggctctggcaagcccggatctggaaaaccaggctccggaaaacctggcagccaggccgtggttacccaagagccttctctgacagtgtctcctggcggcaccgtgacactgacctgtagatcttctaccggcgctgtgaccacctccaactacgccaattgggtgcagcagaagcctggacaggcacccagaggactgatcggaggcaccaacaagagagcccctggcactcctgccagattctctggatctctgctgggcgataaggccgctctgactttgtctggtgcccagcctgaggatgaggctgagtactattgcgccctgtggtactccaacctgtgggttttcggcggtggcaccaaagtgaccgtgctggaacctaagtcctccgacaagacccacacctgtcctccatgtcctgctccagaagctgctggcggcccttccgtgtttctgttccctccaaagcctaaggacaccctgatgatctctcggacccctgaagtgacctgcgtggtggtggatgtgtctcacgaggacccagaagtgaagttcaattggtacgtggacggcgtggaagtgcacaacgccaagaccaagcctagagaggaacagtacggctccacctacagagtggtgtccgtgctgacagtgctgcaccaggattggctgaacggcaaagagtacaagtgcaaggtgtccaacaaggccctgcctgctcctatcgaaaagaccatctccaaggccaagggccagcctagggaaccccaggtttacaccttgcctccaagcagggacgagctgaccaagaaccaggtgtccctgtggtgtctggtcaagggcttctacccctccgatatcgccgtggaatgggagtctaatggccagccagagaacaactacaagacaacccctcctgtgctggactccgacggctcattctttctgtactccaagctgaccgtggacaagtccagatggcagcagggcaacgtgttctcctgcagcgtgatgcacgaggccctgcacaatcactacacacagaagtccctgtctctgtcccctggcaag

SEQ ID NO: 6 - protein, 486 aa, synthetic construct
EVQLVESGGGLIQPGGSLRLSCAASGFTFNTYAMNWVRQAPGKGLEWVARIRSKYNNYATYYADSVKDRFTISRDDSKSTLYLQMNNLRAEDTAVYYCVRHGNFGNSYVSWFAYWGQGTLVTVSSGKPGSGKPGSGKPGSGKPGSQAVVTQEPSLTVSPGGTVTLTCRSSTGAVTTSNYANWVQQKPGQAPRGLIGGTNKRAPGTPARFSGSLLGDKAALTLSGAQPEDEAEYYCALWYSNLWVFGGGTKVTVLEPKSSDKTHTCPPCPAPEAAGGPSVFLFPPKPKDTLMISRTPEVTCVVVDVSHEDPEVKFNWYVDGVEVHNAKTKPREEQYGSTYRVVSVLTVLHQDWLNGKEYKCKVSNKALPAPIEKTISKAKGQPREPQVYTLPPSRDELTKNQVSLWCLVKGFYPSDIAVEWESNGQPENNYKTTPPVLDSDGSFFLYSKLTVDKSRWQQGNVFSCSVMHEALHNHYTQKSLSLSPGK

SEQ ID NO: 7 - DNA, 1353 bp, synthetic construct
  CDS 1..1353: protein_id = 8; translation = QVQLVESGGGVVQPGGSLRLSCAASGFTFSSYGMHWVRQAPGKGLEWVAVIWYDGRNKYYADSVKGRFTISRDNSKNTLYLQMNSLRAEDTAVYYCTRDHSGSGSYYIDYWGQGTLVTVSSASTKGPSVFPLAPSSKSTSGGTAALGCLVKDYFPEPVTVSWNSGALTSGVHTFPAVLQSSGLYSLSSVVTVPSSSLGTQTYICNVNHKPSNTKVDKKVEPKSCDKTHTCPPCPAPEAAGGPSVFLFPPKPKDTLMISRTPEVTCVVVDVSHEDPEVKFNWYVDGVEVHNAKTKPREEQYNSTYRVVSVLTVLHQDWLNGKEYKCKVSNKALAAPIEKTISKAKGQPREPQVYTLPPSRDELTKNQVSLSCAVKGFYPSDIAVEWESNGQPENNYKTTPPVLDSDGSFFLVSKLTVDKSRWQQGNVFSCSVMHEALHNHYTQKSLSLSPGK
  source 1..1353: mol_type = other DNA
caggttcagctggttgaatctggcggcggagttgttcagcctggcggatctctgagactgtcttgtgccgcctccggcttcaccttctcctcttacggaatgcactgggtccgacaggcccctggcaaaggattggaatgggtcgccgtgatttggtacgacggccggaacaagtactacgccgactccgtgaagggcagattcaccatctctcgggacaactccaagaacaccctgtacctgcagatgaactccctgagagccgaggacaccgccgtgtactactgcaccagagatcactccggctccggcagctactacatcgattattggggccagggcaccctggtcaccgtttcttccgctagcaccaagggacccagcgtgttccctctggctccttccagcaagtctacctctggcggaacagctgctctgggctgcctggtcaaggactactttcctgagcctgtgaccgtgtcctggaactctggcgctctgacatctggcgtgcacacctttccagctgtgctgcagtcctccggcctgtactctctgtcctctgtcgtgaccgtgccttccagctctctgggaacccagacctacatctgcaatgtgaaccacaagccttccaacaccaaggtggacaagaaggtggaacccaagtcctgcgacaagacccacacctgtcctccatgtcctgctccagaagctgctggcggcccttccgtgtttctgttccctccaaagcctaaggacaccctgatgatctctcggacccctgaagtgacctgcgtggtggtggatgtgtctcacgaggacccagaagtgaagttcaattggtacgtggacggcgtggaagtgcacaacgccaagaccaagcctagagaggaacagtacaactccacctacagagtggtgtccgtgctgacagtgctgcaccaggattggctgaacggcaaagagtacaagtgcaaggtgtccaacaaggccctggctgctcctatcgaaaagaccatctccaaggccaagggccagcctagggaaccccaggtttacaccttgcctccatctcgggacgagctgaccaagaaccaggtgtccctgtcttgcgctgtgaagggcttctacccctccgatatcgccgtggaatgggagtctaatggccagcctgagaacaactacaagacaacccctcctgtgctggactccgacggctcattcttcctggtgtccaagctgaccgtggacaagtctagatggcagcagggcaacgtgttctcctgcagcgtgatgcacgaggccctgcacaatcactacacacagaagtctctgtctctgagccccggcaag

SEQ ID NO: 8 - protein, 451 aa, synthetic construct
QVQLVESGGGVVQPGGSLRLSCAASGFTFSSYGMHWVRQAPGKGLEWVAVIWYDGRNKYYADSVKGRFTISRDNSKNTLYLQMNSLRAEDTAVYYCTRDHSGSGSYYIDYWGQGTLVTVSSASTKGPSVFPLAPSSKSTSGGTAALGCLVKDYFPEPVTVSWNSGALTSGVHTFPAVLQSSGLYSLSSVVTVPSSSLGTQTYICNVNHKPSNTKVDKKVEPKSCDKTHTCPPCPAPEAAGGPSVFLFPPKPKDTLMISRTPEVTCVVVDVSHEDPEVKFNWYVDGVEVHNAKTKPREEQYNSTYRVVSVLTVLHQDWLNGKEYKCKVSNKALAAPIEKTISKAKGQPREPQVYTLPPSRDELTKNQVSLSCAVKGFYPSDIAVEWESNGQPENNYKTTPPVLDSDGSFFLVSKLTVDKSRWQQGNVFSCSVMHEALHNHYTQKSLSLSPGK

SEQ ID NO: 9 - DNA, 1335 bp, synthetic construct
  CDS 1..1335: protein_id = 10; translation = QVQLQQWGAGLLKPSETLSLTCAVYGGSFSPYYWSWIRQPPGKGLEWIGEINHSGSTNYNPSLKSRVTISVDTSKNQFSLKLSSVTAADTAVYYCARRAGDFDYWGQGTLVTVSSASTKGPSVFPLAPSSKSTSGGTAALGCLVKDYFPEPVTVSWNSGALTSGVHTFPAVLQSSGLYSLSSVVTVPSSSLGTQTYICNVNHKPSNTKVDKKVEPKSCDKTHTCPPCPAPEAAGGPSVFLFPPKPKDTLMISRTPEVTCVVVDVSHEDPEVKFNWYVDGVEVHNAKTKPREEQYNSTYRVVSVLTVLHQDWLNGKEYKCKVSNKALAAPIEKTISKAKGQPREPQVYTLPPSRDELTKNQVSLSCAVKGFYPSDIAVEWESNGQPENNYKTTPPVLDSDGSFFLVSKLTVDKSRWQQGNVFSCSVMHEALHNHYTQKSLSLSPGK
  source 1..1335: mol_type = other DNA
caggttcagttgcagcaatggggcgctggcctgctgaagccttctgagacactgtctctgacctgcgctgtgtacggcggctccttctctccttactactggtcctggatccggcagcctcctggcaaaggactggaatggatcggcgagatcaaccactccggctccaccaactacaaccccagcctgaagtccagagtgaccatctccgtggacacctccaagaaccagttctccctgaagctgtcctccgtgaccgctgctgataccgccgtgtactactgtgctcggagagccggcgacttcgattattggggacagggcacactggtcaccgtgtcctctgctagcaccaagggaccctctgtgttccctctggctccttccagcaagtctacctctggcggaacagctgctctgggctgcctggtcaaggactactttcctgagcctgtgaccgtgtcttggaactctggcgctctgacatctggcgtgcacacctttccagctgtgctgcagtcctccggcctgtactctctgtcctctgtcgtgaccgtgccttccagctctctgggaacccagacctacatctgcaatgtgaaccacaagccttccaacaccaaggtggacaagaaggtggaacccaagtcctgcgacaagacccacacctgtcctccatgtcctgctccagaagctgctggcggcccttccgtgtttctgttccctccaaagcctaaggacaccctgatgatctctcggacccctgaagtgacctgcgtggtggtggatgtgtctcacgaggatcccgaagtgaagttcaattggtacgtggacggcgtggaagtgcacaacgccaagaccaagcctagagaggaacagtacaactccacctacagagtggtgtccgtgctgaccgtgctgcaccaggattggctgaacggcaaagagtacaagtgcaaggtgtccaacaaggccctggccgctcctatcgaaaagaccatcagcaaggccaagggccagcctagggaaccccaggtttacaccttgcctccatctcgggacgagctgaccaagaatcaggtgtccctgtcctgtgccgtgaagggcttctacccttccgatatcgccgtggaatgggagagcaatggccagcctgagaacaactacaagacaacccctcctgtgctggactccgacggctcattcttcctggtgtccaagctgacagtggacaagtccagatggcagcagggcaacgtgttctcctgcagcgtgatgcacgaggccctgcacaatcactacacccagaagagtctgtctctgtcccctggcaag

SEQ ID NO: 10 - protein, 445 aa, synthetic construct
QVQLQQWGAGLLKPSETLSLTCAVYGGSFSPYYWSWIRQPPGKGLEWIGEINHSGSTNYNPSLKSRVTISVDTSKNQFSLKLSSVTAADTAVYYCARRAGDFDYWGQGTLVTVSSASTKGPSVFPLAPSSKSTSGGTAALGCLVKDYFPEPVTVSWNSGALTSGVHTFPAVLQSSGLYSLSSVVTVPSSSLGTQTYICNVNHKPSNTKVDKKVEPKSCDKTHTCPPCPAPEAAGGPSVFLFPPKPKDTLMISRTPEVTCVVVDVSHEDPEVKFNWYVDGVEVHNAKTKPREEQYNSTYRVVSVLTVLHQDWLNGKEYKCKVSNKALAAPIEKTISKAKGQPREPQVYTLPPSRDELTKNQVSLSCAVKGFYPSDIAVEWESNGQPENNYKTTPPVLDSDGSFFLVSKLTVDKSRWQQGNVFSCSVMHEALHNHYTQKSLSLSPGK

SEQ ID NO: 11 - DNA, 636 bp, synthetic construct
  CDS 1..636: protein_id = 12; translation = DIQMTQSPSTLSASVGDRVTITCRASQSISSWLAWYQQKPGKAPKLLIYKASSLESGVPSRFSGSGSGTEFTLTISSLQPDDFATYYCQQYNSYIFGQGTKLEIKRTVAAPSVFIFPPSDEQLKSGTASVVCLLNNFYPREAKVQWKVDNALQSGNSQESVTEQDSKDSTYSLSSTLTLSKADYEKHKVYACEVTHQGLSSPVTKSFNRGEC
  source 1..636: mol_type = other DNA
gacatccagatgacccagtctccatccacactgtccgcctctgtgggcgacagagtgaccatcacctgtcgggcctctcagtccatctcttcttggctggcctggtatcagcagaagcctggcaaggctcccaagctgctgatctacaaggcctcctctctggaatccggcgtgccctctagattctccggctctggatctggcaccgagtttaccctgacaatctccagcctgcagcctgacgacttcgccacctactactgccagcagtacaactcctacatcttcggccagggcaccaagctggaaatcaagcgtacggtggccgctccttccgtgttcatcttcccaccttccgacgagcagctgaagtccggcacagcttctgtcgtgtgcctgctgaacaacttctaccctcgggaagccaaggtgcagtggaaggtggacaatgccctgcagtccggcaactcccaagagtctgtgaccgagcaggactccaaggacagcacctacagcctgtcctccacactgaccctgtccaaggccgactacgagaagcacaaggtgtacgcctgcgaagtgacccatcagggcctgtctagccctgtgaccaagtctttcaaccggggcgagtgc

SEQ ID NO: 12 - protein, 212 aa, synthetic construct
DIQMTQSPSTLSASVGDRVTITCRASQSISSWLAWYQQKPGKAPKLLIYKASSLESGVPSRFSGSGSGTEFTLTISSLQPDDFATYYCQQYNSYIFGQGTKLEIKRTVAAPSVFIFPPSDEQLKSGTASVVCLLNNFYPREAKVQWKVDNALQSGNSQESVTEQDSKDSTYSLSSTLTLSKADYEKHKVYACEVTHQGLSSPVTKSFNRGEC

SEQ ID NO: 13 - DNA, 1458 bp, synthetic construct
  CDS 1..1458: protein_id = 14; translation = EVQLVESGGGLIQPGGSLRLSCAASGFTFNTYAMNWVRQAPGKGLEWVARIRSKYNNYATYYADSVKDRFTISRDDSKSTLYLQMNNLRAEDTAVYYCVRHGNFGDDYVSWFAYWGQGTLVTVSSGKPGSGKPGSGKPGSGKPGSQAVVTQEPSLTVSPGGTVTLTCRSSTGAVTTSNYANWVQQKPGQAPRGLIGGTNKRAPGTPARFSGSLLGDKAALTLSGAQPEDEAEYYCALWYSNLWVFGGGTKVTVLEPKSSDKTHTCPPCPAPEAAGGPSVFLFPPKPKDTLMISRTPEVTCVVVDVSHEDPEVKFNWYVDGVEVHNAKTKPREEQYNSTYRVVSVLTVLHQDWLNGKEYKCKVSNKALAAPIEKTISKAKGQPREPQVYTLPPSRDELTKNQVSLWCLVKGFYPSDIAVEWESNGQPENNYKTTPPVLDSDGSFFLYSKLTVDKSRWQQGNVFSCSVMHEALHNHYTQKSLSLSPGK
  source 1..1458: mol_type = other DNA
gaagtgcagctggttgaatctggcggcggactgattcagcctggcggatctctgagactgtcttgtgccgcctctggcttcaccttcaacacctacgccatgaactgggtccgacaggctcctggcaaaggcctggaatgggtcgcccggatcagatccaagtacaacaattacgccacctactacgccgactccgtgaaggaccggttcaccatctctcgggacgactccaagagcaccctgtacctgcagatgaacaacctgagagccgaggacaccgccgtgtactactgtgtgcggcacggcaacttcggcgacgactatgtgtcttggtttgcctactggggccagggcacactggtcacagtgtcctctggaaagcctggctctggcaagcccggatctggaaaaccaggctccggaaaacctggcagccaggccgtggttacccaagagccttctctgacagtgtctcctggcggcaccgtgacactgacctgtagatcttctaccggcgctgtgaccacctccaactacgccaattgggtgcagcagaagcctggacaggcacccagaggactgatcggaggcaccaacaagagagcccctggcactcctgccagattctctggatctctgctgggcgataaggccgctctgactttgtctggtgcccagcctgaggatgaggctgagtactattgcgccctgtggtactccaacctgtgggttttcggcggtggcaccaaagtgaccgtgctggaacctaagtcctccgacaagacccacacctgtcctccatgtcctgctccagaagctgctggcggcccttccgtgtttctgttccctccaaagcctaaggacaccctgatgatctctcggacccctgaagtgacctgcgtggtggtggatgtgtctcacgaggacccagaagtgaagttcaattggtacgtggacggcgtggaagtgcacaacgccaagaccaagcctagagaggaacagtacaactccacctacagagtggtgtccgtgctgacagtgctgcaccaggattggctgaacggcaaagagtacaagtgcaaggtgtccaacaaggccctggctgctcctatcgaaaagaccatctccaaggccaagggccagcctagggaaccccaggtttacaccttgcctccaagcagggacgagctgaccaagaaccaggtgtccctgtggtgtctggtcaagggcttctacccctccgatatcgccgtggaatgggagtctaatggccagccagagaacaactacaagacaacccctcctgtgctggactccgacggctcattctttctgtactccaagctgaccgtggacaagtccagatggcagcagggcaacgtgttctcctgcagcgtgatgcacgaggccctgcacaatcactacacacagaagtccctgtctctgtcccctggcaag

SEQ ID NO: 14 - protein, 486 aa, synthetic construct
EVQLVESGGGLIQPGGSLRLSCAASGFTFNTYAMNWVRQAPGKGLEWVARIRSKYNNYATYYADSVKDRFTISRDDSKSTLYLQMNNLRAEDTAVYYCVRHGNFGDDYVSWFAYWGQGTLVTVSSGKPGSGKPGSGKPGSGKPGSQAVVTQEPSLTVSPGGTVTLTCRSSTGAVTTSNYANWVQQKPGQAPRGLIGGTNKRAPGTPARFSGSLLGDKAALTLSGAQPEDEAEYYCALWYSNLWVFGGGTKVTVLEPKSSDKTHTCPPCPAPEAAGGPSVFLFPPKPKDTLMISRTPEVTCVVVDVSHEDPEVKFNWYVDGVEVHNAKTKPREEQYNSTYRVVSVLTVLHQDWLNGKEYKCKVSNKALAAPIEKTISKAKGQPREPQVYTLPPSRDELTKNQVSLWCLVKGFYPSDIAVEWESNGQPENNYKTTPPVLDSDGSFFLYSKLTVDKSRWQQGNVFSCSVMHEALHNHYTQKSLSLSPGK

SEQ ID NO: 15 - DNA, 1458 bp, synthetic construct
  CDS 1..1458: protein_id = 16; translation = EVQLVESGGGLIQPGGSLRLSCAASGFTFNTYAMNWVRQAPGKGLEWVARIRSKYNNYATEYADSVKDRFTISRDDSKSTLYLQMNNLRAEDTAVYYCVRHGNFGNSYVSWFAYWGQGTLVTVSSGKPGSGKPGSGKPGSGKPGSQAVVTQEPSLTVSPGGTVTLTCRSSTGAVTTSNYANWVQQKPGQAPRGLIGGTNKRAPGTPARFSGSLLGDKAALTISGAQPEDEAEYYCALWYSNLWVFGGGTKVTVLEPKSSDKTHTCPPCPAPEAAGGPSVFLFPPKPKDTLMISRTPEVTCVVVDVSHEDPEVKFNWYVDGVEVHNAKTKPREEQYNSTYRVVSVLTVLHQDWLNGKEYKCKVSNKALAAPIEKTISKAKGQPREPQVYTLPPSRDELTKNQVSLWCLVKGFYPSDIAVEWESNGQPENNYKTTPPVLDSDGSFFLYSKLTVDKSRWQQGNVFSCSVMHEALHNHYTQKSLSLSPGK
  source 1..1458: mol_type = other DNA
gaagtgcagctggttgaatctggcggcggactgattcagcctggcggatctctgagactgtcttgtgccgcctctggcttcaccttcaacacctacgccatgaactgggtccgacaggctcctggcaaaggcctggaatgggtcgcccggatcagatccaagtacaacaattacgccaccgagtacgccgactccgtgaaggacagattcaccatctctcgggacgactccaagagcaccctgtacctgcagatgaacaacctgagagccgaggacaccgccgtgtactactgtgtgcggcacggcaacttcggcaactcctatgtgtcttggtttgcctactggggccagggcacactggtcacagtgtcctctggaaagcctggctctggcaagcccggatctggaaaaccaggctccggaaaacctggcagccaggccgtggttacccaagagccttctctgacagtgtctcctggcggcaccgtgacactgacctgtagatcttctaccggcgctgtgaccacctccaactacgccaattgggtgcagcagaagcctggacaggcacccagaggactgatcggaggcaccaacaagagagcccctggcactcctgccagattctctggatctctgctgggcgataaggccgctctgactatctctggtgcccagcctgaggatgaggctgagtactattgcgccctgtggtactccaacctgtgggttttcggcggtggcaccaaagtgaccgtgctggaacctaagtcctccgacaagacccacacctgtcctccatgtcctgctccagaagctgctggcggcccttccgtgtttctgttccctccaaagcctaaggacaccctgatgatctctcggacccctgaagtgacctgcgtggtggtggatgtgtctcacgaggacccagaagtgaagttcaattggtacgtggacggcgtggaagtgcacaacgccaagaccaagcctagagaggaacagtacaactccacctacagagtggtgtccgtgctgacagtgctgcaccaggattggctgaacggcaaagagtacaagtgcaaggtgtccaacaaggccctggctgctcctatcgaaaagaccatctccaaggccaagggccagcctagggaaccccaggtttacaccttgcctccaagcagggacgagctgaccaagaaccaggtgtccctgtggtgtctggtcaagggcttctacccctccgatatcgccgtggaatgggagtctaatggccagccagagaacaactacaagacaacccctcctgtgctggactccgacggctcattctttctgtactccaagctgaccgtggacaagtccagatggcagcagggcaacgtgttctcctgcagcgtgatgcacgaggccctgcacaatcactacacacagaagtccctgtctctgtcccctggcaag

SEQ ID NO: 16 - protein, 486 aa, synthetic construct
EVQLVESGGGLIQPGGSLRLSCAASGFTFNTYAMNWVRQAPGKGLEWVARIRSKYNNYATEYADSVKDRFTISRDDSKSTLYLQMNNLRAEDTAVYYCVRHGNFGNSYVSWFAYWGQGTLVTVSSGKPGSGKPGSGKPGSGKPGSQAVVTQEPSLTVSPGGTVTLTCRSSTGAVTTSNYANWVQQKPGQAPRGLIGGTNKRAPGTPARFSGSLLGDKAALTISGAQPEDEAEYYCALWYSNLWVFGGGTKVTVLEPKSSDKTHTCPPCPAPEAAGGPSVFLFPPKPKDTLMISRTPEVTCVVVDVSHEDPEVKFNWYVDGVEVHNAKTKPREEQYNSTYRVVSVLTVLHQDWLNGKEYKCKVSNKALAAPIEKTISKAKGQPREPQVYTLPPSRDELTKNQVSLWCLVKGFYPSDIAVEWESNGQPENNYKTTPPVLDSDGSFFLYSKLTVDKSRWQQGNVFSCSVMHEALHNHYTQKSLSLSPGK

SEQ ID NO: 17 - DNA, 1458 bp, synthetic construct
  CDS 1..1458: protein_id = 18; translation = EVQLVESGGGLIQPGGSLRLSCAASGFTFNTYAMNWVRQAPGKGLEWVARIRSKYNNYATYYADSVKDRFTISRDDSKSTLYLQMNNLRAEDTAVYYCVRHGNFGNDYVSWFAYWGQGTLVTVSSGKPGSGKPGSGKPGSGKPGSQAVVTQEPSLTVSPGGTVTLTCRSSTGAVTTSNYANWVQQKPGQAPRGLIGGTNKRAPGTPARFSGSLLGDKAALTLSGAQPEDEADYYCALWYSNLWVFGGGTKVTVLEPKSSDKTHTCPPCPAPEAAGGPSVFLFPPKPKDTLMISRTPEVTCVVVDVSHEDPEVKFNWYVDGVEVHNAKTKPREEQYNSTYRVVSVLTVLHQDWLNGKEYKCKVSNKALAAPIEKTISKAKGQPREPQVYTLPPSRDELTKNQVSLWCLVKGFYPSDIAVEWESNGQPENNYKTTPPVLDSDGSFFLYSKLTVDKSRWQQGNVFSCSVMHEALHNHYTQKSLSLSPGK
  source 1..1458: mol_type = other DNA
gaagtgcagctggttgaatctggcggcggactgattcagcctggcggatctctgagactgtcttgtgccgcctctggcttcaccttcaacacctacgccatgaactgggtccgacaggctcctggcaaaggcctggaatgggtcgcccggatcagatccaagtacaacaattacgccacctactacgccgactccgtgaaggaccggttcaccatctctcgggacgactccaagagcaccctgtacctgcagatgaacaacctgagagccgaggacaccgccgtgtactactgtgtgcggcacggcaacttcggcaacgactatgtgtcttggtttgcctactggggccagggcacactggtcacagtgtcctctggaaagcctggctctggcaagcccggatctggaaaaccaggctccggaaaacctggcagccaggccgtggttacccaagagccttctctgacagtgtctcctggcggcaccgtgacactgacctgtagatcttctaccggcgctgtgaccacctccaactacgccaattgggtgcagcagaagcctggacaggcacccagaggactgatcggaggcaccaacaagagagcccctggcactcctgccagattctctggatctctgctgggcgataaggccgctctgactttgtctggtgcccagcctgaggatgaggctgattactattgcgccctgtggtactccaacctgtgggttttcggcggtggcaccaaagtgaccgtgctggaacctaagtcctccgacaagacccacacctgtcctccatgtcctgctccagaagctgctggcggcccttccgtgtttctgttccctccaaagcctaaggacaccctgatgatctctcggacccctgaagtgacctgcgtggtggtggatgtgtctcacgaggacccagaagtgaagttcaattggtacgtggacggcgtggaagtgcacaacgccaagaccaagcctagagaggaacagtacaactccacctacagagtggtgtccgtgctgacagtgctgcaccaggattggctgaacggcaaagagtacaagtgcaaggtgtccaacaaggccctggctgctcctatcgaaaagaccatctccaaggccaagggccagcctagggaaccccaggtttacaccttgcctccaagcagggacgagctgaccaagaaccaggtgtccctgtggtgtctggtcaagggcttctacccctccgatatcgccgtggaatgggagtctaatggccagccagagaacaactacaagacaacccctcctgtgctggactccgacggctcattctttctgtactccaagctgaccgtggacaagtccagatggcagcagggcaacgtgttctcctgcagcgtgatgcacgaggccctgcacaatcactacacacagaagtccctgtctctgtcccctggcaag

SEQ ID NO: 18 - protein, 486 aa, synthetic construct
EVQLVESGGGLIQPGGSLRLSCAASGFTFNTYAMNWVRQAPGKGLEWVARIRSKYNNYATYYADSVKDRFTISRDDSKSTLYLQMNNLRAEDTAVYYCVRHGNFGNDYVSWFAYWGQGTLVTVSSGKPGSGKPGSGKPGSGKPGSQAVVTQEPSLTVSPGGTVTLTCRSSTGAVTTSNYANWVQQKPGQAPRGLIGGTNKRAPGTPARFSGSLLGDKAALTLSGAQPEDEADYYCALWYSNLWVFGGGTKVTVLEPKSSDKTHTCPPCPAPEAAGGPSVFLFPPKPKDTLMISRTPEVTCVVVDVSHEDPEVKFNWYVDGVEVHNAKTKPREEQYNSTYRVVSVLTVLHQDWLNGKEYKCKVSNKALAAPIEKTISKAKGQPREPQVYTLPPSRDELTKNQVSLWCLVKGFYPSDIAVEWESNGQPENNYKTTPPVLDSDGSFFLYSKLTVDKSRWQQGNVFSCSVMHEALHNHYTQKSLSLSPGK

SEQ ID NO: 19 - DNA, 1458 bp, synthetic construct
  CDS 1..1458: protein_id = 20; translation = EVQLVESGGGLIQPGGSLRLSCAASGFTFNTYAMNWVRQAPGKGLEWVARIRSKYNNYATYYADSVKDRFTISRDDSKSTLYLQMNNLRAEDTAVYYCVRHGNFGDSYVSWFDYWGQGTLVTVSSGKPGSGKPGSGKPGSGKPGSQAVVTQEPSLTVSPGGTVTLTCRSSTGAVTTSNYANWVQQKPGQAPRGLIGGTNKRAPGTPARFSGSLLGDKAALTLSGAQPEDEAEYYCALWYSNLWVFGGGTKVTVLEPKSSDKTHTCPPCPAPEAAGGPSVFLFPPKPKDTLMISRTPEVTCVVVDVSHEDPEVKFNWYVDGVEVHNAKTKPREEQYNSTYRVVSVLTVLHQDWLNGKEYKCKVSNKALAAPIEKTISKAKGQPREPQVYTLPPSRDELTKNQVSLWCLVKGFYPSDIAVEWESNGQPENNYKTTPPVLDSDGSFFLYSKLTVDKSRWQQGNVFSCSVMHEALHNHYTQKSLSLSPGK
  source 1..1458: mol_type = other DNA
gaagtgcagctggttgaatctggcggcggactgattcagcctggcggatctctgagactgtcttgtgccgcctctggcttcaccttcaacacctacgccatgaactgggtccgacaggctcctggcaaaggcctggaatgggtcgcccggatcagatccaagtacaacaattacgccacctactacgccgactccgtgaaggaccggttcaccatctctcgggacgactccaagagcaccctgtacctgcagatgaacaacctgagagccgaggacaccgccgtgtactactgtgtgcggcacggcaacttcggcgactcctatgtgtcttggtttgactactggggccagggcaccctggtcacagtgtcctctggaaagcctggctctggcaagcccggatctggaaaaccaggctccggaaaacctggcagccaggccgtggttacccaagagccttctctgacagtgtctcctggcggcaccgtgacactgacctgtagatcttctaccggcgctgtgaccacctccaactacgccaattgggtgcagcagaagcctggacaggcacccagaggactgatcggaggcaccaacaagagagcccctggcactcctgccagattctctggatctctgctgggcgataaggccgctctgactttgtctggtgcccagcctgaggatgaggctgagtactattgcgccctgtggtactccaacctgtgggttttcggcggtggcaccaaagtgaccgtgctggaacctaagtcctccgacaagacccacacctgtcctccatgtcctgctccagaagctgctggcggcccttccgtgtttctgttccctccaaagcctaaggacaccctgatgatctctcggacccctgaagtgacctgcgtggtggtggatgtgtctcacgaggacccagaagtgaagttcaattggtacgtggacggcgtggaagtgcacaacgccaagaccaagcctagagaggaacagtacaactccacctacagagtggtgtccgtgctgacagtgctgcaccaggattggctgaacggcaaagagtacaagtgcaaggtgtccaacaaggccctggctgctcctatcgaaaagaccatctccaaggccaagggccagcctagggaaccccaggtttacaccttgcctccaagcagggacgagctgaccaagaaccaggtgtccctgtggtgtctggtcaagggcttctacccctccgatatcgccgtggaatgggagtctaatggccagccagagaacaactacaagacaacccctcctgtgctggactccgacggctcattctttctgtactccaagctgaccgtggacaagtccagatggcagcagggcaacgtgttctcctgcagcgtgatgcacgaggccctgcacaatcactacacacagaagtccctgtctctgtcccctggcaag

SEQ ID NO: 20 - protein, 486 aa, synthetic construct
EVQLVESGGGLIQPGGSLRLSCAASGFTFNTYAMNWVRQAPGKGLEWVARIRSKYNNYATYYADSVKDRFTISRDDSKSTLYLQMNNLRAEDTAVYYCVRHGNFGDSYVSWFDYWGQGTLVTVSSGKPGSGKPGSGKPGSGKPGSQAVVTQEPSLTVSPGGTVTLTCRSSTGAVTTSNYANWVQQKPGQAPRGLIGGTNKRAPGTPARFSGSLLGDKAALTLSGAQPEDEAEYYCALWYSNLWVFGGGTKVTVLEPKSSDKTHTCPPCPAPEAAGGPSVFLFPPKPKDTLMISRTPEVTCVVVDVSHEDPEVKFNWYVDGVEVHNAKTKPREEQYNSTYRVVSVLTVLHQDWLNGKEYKCKVSNKALAAPIEKTISKAKGQPREPQVYTLPPSRDELTKNQVSLWCLVKGFYPSDIAVEWESNGQPENNYKTTPPVLDSDGSFFLYSKLTVDKSRWQQGNVFSCSVMHEALHNHYTQKSLSLSPGK

SEQ ID NO: 21 - DNA, 1458 bp, synthetic construct
  CDS 1..1458: protein_id = 22; translation = EVQLVESGGGLIQPGGSLRLSCAASGFTFNTYAMNWVRQAPGKGLEWVARIRSKYNNYATYYADSVKDRFTISRDDSKSTLYLQMNNLRAEDTAVYYCVRHGNFGNDYVSWFAYWGQGTLVTVSSGKPGSGKPGSGKPGSGKPGSQAVVTQEPSLTVSPGGTVTLTCRSSTGAVTTSNYANWVQQKPGQAPRGLIGGTNKRAPGVPARFSGSLLGDKAALTLSGAQPEDEAEYYCALWYSNLWVFGGGTKVTVLEPKSSDKTHTCPPCPAPEAAGGPSVFLFPPKPKDTLMISRTPEVTCVVVDVSHEDPEVKFNWYVDGVEVHNAKTKPREEQYNSTYRVVSVLTVLHQDWLNGKEYKCKVSNKALAAPIEKTISKAKGQPREPQVYTLPPSRDELTKNQVSLWCLVKGFYPSDIAVEWESNGQPENNYKTTPPVLDSDGSFFLYSKLTVDKSRWQQGNVFSCSVMHEALHNHYTQKSLSLSPGK
  source 1..1458: mol_type = other DNA
gaagtgcagctggttgaatctggcggcggactgattcagcctggcggatctctgagactgtcttgtgccgcctctggcttcaccttcaacacctacgccatgaactgggtccgacaggctcctggcaaaggcctggaatgggtcgcccggatcagatccaagtacaacaattacgccacctactacgccgactccgtgaaggaccggttcaccatctctcgggacgactccaagagcaccctgtacctgcagatgaacaacctgagagccgaggacaccgccgtgtactactgtgtgcggcacggcaacttcggcaacgactatgtgtcttggtttgcctactggggccagggcacactggtcacagtgtcctctggaaagcctggctctggcaagcccggatctggaaaaccaggctccggaaaacctggcagccaggccgtggttacccaagagccttctctgacagtgtctcctggcggcaccgtgacactgacctgtagatcttctaccggcgctgtgaccacctccaactacgccaattgggtgcagcagaagcctggacaggcacccagaggactgatcggaggcaccaacaagagagcccctggcgtgcctgccagattctctggatctctgctgggcgataaggccgctctgactttgtctggtgcccagcctgaggatgaggctgagtactattgcgccctgtggtactccaacctgtgggttttcggcggtggcaccaaagtgaccgtgctggaacctaagtcctccgacaagacccacacctgtcctccatgtcctgctccagaagctgctggcggcccttccgtgtttctgttccctccaaagcctaaggacaccctgatgatctctcggacccctgaagtgacctgcgtggtggtggatgtgtctcacgaggacccagaagtgaagttcaattggtacgtggacggcgtggaagtgcacaacgccaagaccaagcctagagaggaacagtacaactccacctacagagtggtgtccgtgctgacagtgctgcaccaggattggctgaacggcaaagagtacaagtgcaaggtgtccaacaaggccctggctgctcctatcgaaaagaccatctccaaggccaagggccagcctagggaaccccaggtttacaccttgcctccaagcagggacgagctgaccaagaaccaggtgtccctgtggtgtctggtcaagggcttctacccctccgatatcgccgtggaatgggagtctaatggccagccagagaacaactacaagacaacccctcctgtgctggactccgacggctcattctttctgtactccaagctgaccgtggacaagtccagatggcagcagggcaacgtgttctcctgcagcgtgatgcacgaggccctgcacaatcactacacacagaagtccctgtctctgtcccctggcaag

SEQ ID NO: 22 - protein, 486 aa, synthetic construct
EVQLVESGGGLIQPGGSLRLSCAASGFTFNTYAMNWVRQAPGKGLEWVARIRSKYNNYATYYADSVKDRFTISRDDSKSTLYLQMNNLRAEDTAVYYCVRHGNFGNDYVSWFAYWGQGTLVTVSSGKPGSGKPGSGKPGSGKPGSQAVVTQEPSLTVSPGGTVTLTCRSSTGAVTTSNYANWVQQKPGQAPRGLIGGTNKRAPGVPARFSGSLLGDKAALTLSGAQPEDEAEYYCALWYSNLWVFGGGTKVTVLEPKSSDKTHTCPPCPAPEAAGGPSVFLFPPKPKDTLMISRTPEVTCVVVDVSHEDPEVKFNWYVDGVEVHNAKTKPREEQYNSTYRVVSVLTVLHQDWLNGKEYKCKVSNKALAAPIEKTISKAKGQPREPQVYTLPPSRDELTKNQVSLWCLVKGFYPSDIAVEWESNGQPENNYKTTPPVLDSDGSFFLYSKLTVDKSRWQQGNVFSCSVMHEALHNHYTQKSLSLSPGK

SEQ ID NO: 23 - DNA, 1458 bp, synthetic construct
  CDS 1..1458: protein_id = 24; translation = EVQLVESGGGLIQPGGSLRLSCAASGFTFNTYAMNWVRQAPGKGLEWVARIRSKYNNYATYYADSVKDRFTISRDDSKSTLYLQMNNLRAEDTAVYYCVRHGNFGNSYVSWFDYWGQGTLVTVSSGKPGSGKPGSGKPGSGKPGSQAVVTQEPSLTVSPGGTVTLTCRSSTGAVTTSNYANWVQQKPGQAPRGLIGGTNKRAPGVPARFSGSLLGDKAALTLSGAQPEDEAEYYCALWYSNLWVFGGGTKVTVLEPKSSDKTHTCPPCPAPEAAGGPSVFLFPPKPKDTLMISRTPEVTCVVVDVSHEDPEVKFNWYVDGVEVHNAKTKPREEQYNSTYRVVSVLTVLHQDWLNGKEYKCKVSNKALAAPIEKTISKAKGQPREPQVYTLPPSRDELTKNQVSLWCLVKGFYPSDIAVEWESNGQPENNYKTTPPVLDSDGSFFLYSKLTVDKSRWQQGNVFSCSVMHEALHNHYTQKSLSLSPGK
  source 1..1458: mol_type = other DNA
gaagtgcagctggttgaatctggcggcggactgattcagcctggcggatctctgagactgtcttgtgccgcctctggcttcaccttcaacacctacgccatgaactgggtccgacaggctcctggcaaaggcctggaatgggtcgcccggatcagatccaagtacaacaattacgccacctactacgccgactccgtgaaggaccggttcaccatctctcgggacgactccaagagcaccctgtacctgcagatgaacaacctgagagccgaggacaccgccgtgtactactgtgtgcggcacggcaacttcggcaactcctatgtgtcttggtttgactactggggccagggcaccctggtcacagtgtcctctggaaagcctggctctggcaagcccggatctggaaaaccaggctccggaaaacctggcagccaggccgtggttacccaagagccttctctgacagtgtctcctggcggcaccgtgacactgacctgtagatcttctaccggcgctgtgaccacctccaactacgccaattgggtgcagcagaagcctggacaggcacccagaggactgatcggaggcaccaacaagagagcccctggcgtgcctgccagattctctggatctctgctgggcgataaggccgctctgactttgtctggtgcccagcctgaggatgaggctgagtactattgcgccctgtggtactccaacctgtgggttttcggcggtggcaccaaagtgaccgtgctggaacctaagtcctccgacaagacccacacctgtcctccatgtcctgctccagaagctgctggcggcccttccgtgtttctgttccctccaaagcctaaggacaccctgatgatctctcggacccctgaagtgacctgcgtggtggtggatgtgtctcacgaggacccagaagtgaagttcaattggtacgtggacggcgtggaagtgcacaacgccaagaccaagcctagagaggaacagtacaactccacctacagagtggtgtccgtgctgacagtgctgcaccaggattggctgaacggcaaagagtacaagtgcaaggtgtccaacaaggccctggctgctcctatcgaaaagaccatctccaaggccaagggccagcctagggaaccccaggtttacaccttgcctccaagcagggacgagctgaccaagaaccaggtgtccctgtggtgtctggtcaagggcttctacccctccgatatcgccgtggaatgggagtctaatggccagccagagaacaactacaagacaacccctcctgtgctggactccgacggctcattctttctgtactccaagctgaccgtggacaagtccagatggcagcagggcaacgtgttctcctgcagcgtgatgcacgaggccctgcacaatcactacacacagaagtccctgtctctgtcccctggcaag

SEQ ID NO: 24 - protein, 486 aa, synthetic construct
EVQLVESGGGLIQPGGSLRLSCAASGFTFNTYAMNWVRQAPGKGLEWVARIRSKYNNYATYYADSVKDRFTISRDDSKSTLYLQMNNLRAEDTAVYYCVRHGNFGNSYVSWFDYWGQGTLVTVSSGKPGSGKPGSGKPGSGKPGSQAVVTQEPSLTVSPGGTVTLTCRSSTGAVTTSNYANWVQQKPGQAPRGLIGGTNKRAPGVPARFSGSLLGDKAALTLSGAQPEDEAEYYCALWYSNLWVFGGGTKVTVLEPKSSDKTHTCPPCPAPEAAGGPSVFLFPPKPKDTLMISRTPEVTCVVVDVSHEDPEVKFNWYVDGVEVHNAKTKPREEQYNSTYRVVSVLTVLHQDWLNGKEYKCKVSNKALAAPIEKTISKAKGQPREPQVYTLPPSRDELTKNQVSLWCLVKGFYPSDIAVEWESNGQPENNYKTTPPVLDSDGSFFLYSKLTVDKSRWQQGNVFSCSVMHEALHNHYTQKSLSLSPGK

SEQ ID NO: 25 - DNA, 1458 bp, synthetic construct
  source 1..1458: mol_type = other DNA
  CDS 1..1458: protein_id = 26; translation = EVQLVESGGGLIQPGGSLRLSCAASGFTFSDHAMNWVRQAPGKGLEWVARIRSKYNNYATYYADSVKDRFTISRDDSKSTLYLQMNNLRAEDTAVYYCVRHGNFGNSYVSWFAYWGQGTLVTVSSGKPGSGKPGSGKPGSGKPGSQAVVTQEPSLTVSPGGTVTLTCRSSTGAVTTSNYANWVQQKPGQAPRGLIGGTNKRAPGTPARFSGSLLGDKAALTISGAQPEDEAEYYCALWYSNLWVFGGGTKVTVLEPKSSDKTHTCPPCPAPEAAGGPSVFLFPPKPKDTLMISRTPEVTCVVVDVSHEDPEVKFNWYVDGVEVHNAKTKPREEQYNSTYRVVSVLTVLHQDWLNGKEYKCKVSNKALAAPIEKTISKAKGQPREPQVYTLPPSRDELTKNQVSLWCLVKGFYPSDIAVEWESNGQPENNYKTTPPVLDSDGSFFLYSKLTVDKSRWQQGNVFSCSVMHEALHNHYTQKSLSLSPGK
gaagtgcagctggttgaatctggcggcggactgattcagcctggcggatctctgagactgtcttgtgccgcctctggcttcaccttctctgaccacgccatgaactgggtccgacaggctcctggcaaaggcctggaatgggtcgcccggatcagatccaagtacaacaactacgccacctactacgccgactccgtgaaggaccggttcaccatctctcgggacgactccaagagcaccctgtacctgcagatgaacaacctgagagccgaggacaccgccgtgtactactgtgtgcggcacggcaacttcggcaactcctatgtgtcttggtttgcctactggggccagggcacactggtcacagtgtcctctggaaagcctggctctggcaagcccggatctggaaaaccaggctccggaaaacctggcagccaggccgtggttacccaagagcctagtctgacagtgtctcctggcggcaccgtgacactgacctgtagatcttctaccggcgctgtgaccacctccaattacgccaattgggtgcagcagaagcccggccaagctcctagaggactgatcggaggcaccaacaagagagcccctggcactcctgccagattctctggatctctgctgggcgataaggccgctctgacaatctctggtgcccagcctgaggatgaggctgagtactattgcgccctgtggtactccaacctgtgggttttcggcggtggcaccaaagtgaccgtgctggaacctaagtcctccgacaagacccacacctgtcctccatgtcctgctccagaagctgctggcggcccttccgtgtttctgttccctccaaagcctaaggacaccctgatgatctctcggacccctgaagtgacctgcgtggtggtggatgtgtctcacgaggacccagaagtgaagttcaattggtacgtggacggcgtggaagtgcacaacgccaagaccaagcctagagaggaacagtacaactccacctacagagtggtgtccgtgctgacagtgctgcaccaggattggctgaacggcaaagagtacaagtgcaaggtgtccaacaaggccctggctgctcctatcgaaaagaccatctccaaggccaagggccagcctagggaaccccaggtttacaccttgcctccaagcagggacgagctgaccaagaaccaggtgtccctgtggtgtctggtcaagggcttctacccctccgatatcgccgtggaatgggagtctaatggccagccagagaacaactacaagacaacccctcctgtgctggactccgacggctcattctttctgtactccaagctgaccgtggacaagtccagatggcagcagggcaacgtgttctcctgcagcgtgatgcacgaggccctgcacaatcactacacacagaagtccctgtctctgtcccctggcaag

SEQ ID NO: 26 - protein, 486 aa, synthetic construct
EVQLVESGGGLIQPGGSLRLSCAASGFTFSDHAMNWVRQAPGKGLEWVARIRSKYNNYATYYADSVKDRFTISRDDSKSTLYLQMNNLRAEDTAVYYCVRHGNFGNSYVSWFAYWGQGTLVTVSSGKPGSGKPGSGKPGSGKPGSQAVVTQEPSLTVSPGGTVTLTCRSSTGAVTTSNYANWVQQKPGQAPRGLIGGTNKRAPGTPARFSGSLLGDKAALTISGAQPEDEAEYYCALWYSNLWVFGGGTKVTVLEPKSSDKTHTCPPCPAPEAAGGPSVFLFPPKPKDTLMISRTPEVTCVVVDVSHEDPEVKFNWYVDGVEVHNAKTKPREEQYNSTYRVVSVLTVLHQDWLNGKEYKCKVSNKALAAPIEKTISKAKGQPREPQVYTLPPSRDELTKNQVSLWCLVKGFYPSDIAVEWESNGQPENNYKTTPPVLDSDGSFFLYSKLTVDKSRWQQGNVFSCSVMHEALHNHYTQKSLSLSPGK

SEQ ID NO: 27 - DNA, 1458 bp, synthetic construct
  CDS 1..1458: protein_id = 28; translation = EVQLVESGGGLIQPGGSLRLSCAASGFTFNTYAMNWVRQAPGKGLEWVARIRSKANNYATYYADSVKDRFTISRDDSKSTLYLQMNNLRAEDTAVYYCVRHGNFGNSYVSWFAYWGQGTLVTVSSGKPGSGKPGSGKPGSGKPGSQAVVTQEPSLTVSPGGTVTLTCRSSTGAVTTSNYANWVQQKPGQAPRGLIGGTNKRAPGTPARFSGSLLGDKAALTISGAQPEDEAEYYCALWYSNLWVFGGGTKVTVLEPKSSDKTHTCPPCPAPEAAGGPSVFLFPPKPKDTLMISRTPEVTCVVVDVSHEDPEVKFNWYVDGVEVHNAKTKPREEQYNSTYRVVSVLTVLHQDWLNGKEYKCKVSNKALAAPIEKTISKAKGQPREPQVYTLPPSRDELTKNQVSLWCLVKGFYPSDIAVEWESNGQPENNYKTTPPVLDSDGSFFLYSKLTVDKSRWQQGNVFSCSVMHEALHNHYTQKSLSLSPGK
  source 1..1458: mol_type = other DNA
gaagtgcagctggttgaatctggcggcggactgattcagcctggcggatctctgagactgtcttgtgccgcctctggcttcaccttcaacacctacgccatgaactgggtccgacaggctcctggcaaaggcctggaatgggtcgcccggatcagatccaaggccaacaattacgccacctactacgccgactccgtgaaggaccggttcaccatctctcgggacgactccaagagcaccctgtacctgcagatgaacaacctgagagccgaggacaccgccgtgtactactgtgtgcggcacggcaacttcggcaactcctatgtgtcttggtttgcctactggggccagggcacactggtcacagtgtcctctggaaagcctggctctggcaagcccggatctggaaaaccaggctccggaaaacctggcagccaggccgtggttacccaagagccttctctgacagtgtctcctggcggcaccgtgacactgacctgtagatcttctaccggcgctgtgaccacctccaactacgccaattgggtgcagcagaagcctggacaggcacccagaggactgatcggaggcaccaacaagagagcccctggcactcctgccagattctctggatctctgctgggcgataaggccgctctgactatctctggtgcccagcctgaggatgaggctgagtactattgcgccctgtggtactccaacctgtgggttttcggcggtggcaccaaagtgaccgtgctggaacctaagtcctccgacaagacccacacctgtcctccatgtcctgctccagaagctgctggcggcccttccgtgtttctgttccctccaaagcctaaggacaccctgatgatctctcggacccctgaagtgacctgcgtggtggtggatgtgtctcacgaggacccagaagtgaagttcaattggtacgtggacggcgtggaagtgcacaacgccaagaccaagcctagagaggaacagtacaactccacctacagagtggtgtccgtgctgacagtgctgcaccaggattggctgaacggcaaagagtacaagtgcaaggtgtccaacaaggccctggctgctcctatcgaaaagaccatcagcaaggccaagggccagcctagggaaccccaggtttacaccttgcctccaagcagggacgagctgaccaagaaccaggtgtccctgtggtgtctggtcaagggcttctacccctccgatatcgccgtggaatgggagtctaatggccagccagagaacaactacaagacaacccctcctgtgctggactccgacggctcattctttctgtactccaagctgaccgtggacaagtccagatggcagcagggcaacgtgttctcctgcagcgtgatgcacgaggccctgcacaatcactacacacagaagtccctgtctctgtcccctggcaag

SEQ ID NO: 28 - protein, 486 aa, synthetic construct
EVQLVESGGGLIQPGGSLRLSCAASGFTFNTYAMNWVRQAPGKGLEWVARIRSKANNYATYYADSVKDRFTISRDDSKSTLYLQMNNLRAEDTAVYYCVRHGNFGNSYVSWFAYWGQGTLVTVSSGKPGSGKPGSGKPGSGKPGSQAVVTQEPSLTVSPGGTVTLTCRSSTGAVTTSNYANWVQQKPGQAPRGLIGGTNKRAPGTPARFSGSLLGDKAALTISGAQPEDEAEYYCALWYSNLWVFGGGTKVTVLEPKSSDKTHTCPPCPAPEAAGGPSVFLFPPKPKDTLMISRTPEVTCVVVDVSHEDPEVKFNWYVDGVEVHNAKTKPREEQYNSTYRVVSVLTVLHQDWLNGKEYKCKVSNKALAAPIEKTISKAKGQPREPQVYTLPPSRDELTKNQVSLWCLVKGFYPSDIAVEWESNGQPENNYKTTPPVLDSDGSFFLYSKLTVDKSRWQQGNVFSCSVMHEALHNHYTQKSLSLSPGK

SEQ ID NO: 29 - DNA, 1458 bp, synthetic construct
  CDS 1..1458: protein_id = 30; translation = EVQLVESGGGLIQPGGSLRLSCAASGFTFNTYAMNWVRQAPGKGLEWVARIRSKYNNYATSYADSVKDRFTISRDDSKSTLYLQMNNLRAEDTAVYYCVRHGNFGNSYVSWFAYWGQGTLVTVSSGKPGSGKPGSGKPGSGKPGSQAVVTQEPSLTVSPGGTVTLTCRSSTGAVTTSNYANWVQQKPGQAPRGLIGGTNKRAPGTPARFSGSLLGDKAALTISGAQPEDEAEYYCALWYSNLWVFGGGTKVTVLEPKSSDKTHTCPPCPAPEAAGGPSVFLFPPKPKDTLMISRTPEVTCVVVDVSHEDPEVKFNWYVDGVEVHNAKTKPREEQYNSTYRVVSVLTVLHQDWLNGKEYKCKVSNKALAAPIEKTISKAKGQPREPQVYTLPPSRDELTKNQVSLWCLVKGFYPSDIAVEWESNGQPENNYKTTPPVLDSDGSFFLYSKLTVDKSRWQQGNVFSCSVMHEALHNHYTQKSLSLSPGK
  source 1..1458: mol_type = other DNA
gaagtgcagctggttgaatctggcggcggactgattcagcctggcggatctctgagactgtcttgtgccgcctctggcttcaccttcaacacctacgccatgaactgggtccgacaggctcctggcaaaggcctggaatgggtcgcccggatcagatccaagtacaacaattacgccacctcctacgccgactccgtgaaggacagattcaccatctctcgggacgactccaagagcaccctgtacctgcagatgaacaacctgagagccgaggacaccgccgtgtactactgtgtgcggcacggcaacttcggcaactcctatgtgtcttggtttgcctactggggccagggcacactggtcacagtgtcctctggaaagcctggctctggcaagcccggatctggaaaaccaggctccggaaaacctggcagccaggccgtggttacccaagagccttctctgacagtgtctcctggcggcaccgtgacactgacctgtagatcttctaccggcgctgtgaccacctccaactacgccaattgggtgcagcagaagcctggacaggcacccagaggactgatcggaggcaccaacaagagagcccctggcactcctgccagattctctggatctctgctgggcgataaggccgctctgactatctctggtgcccagcctgaggatgaggctgagtactattgcgccctgtggtactccaacctgtgggttttcggcggtggcaccaaagtgaccgtgctggaacctaagtcctccgacaagacccacacctgtcctccatgtcctgctccagaagctgctggcggcccttccgtgtttctgttccctccaaagcctaaggacaccctgatgatctctcggacccctgaagtgacctgcgtggtggtggatgtgtctcacgaggacccagaagtgaagttcaattggtacgtggacggcgtggaagtgcacaacgccaagaccaagcctagagaggaacagtacaactccacctacagagtggtgtccgtgctgacagtgctgcaccaggattggctgaacggcaaagagtacaagtgcaaggtgtccaacaaggccctggctgctcctatcgaaaagaccatctccaaggccaagggccagcctagggaaccccaggtttacaccttgcctccaagcagggacgagctgaccaagaaccaggtgtccctgtggtgtctggtcaagggcttctacccctccgatatcgccgtggaatgggagtctaatggccagccagagaacaactacaagacaacccctcctgtgctggactccgacggctcattctttctgtactccaagctgaccgtggacaagtccagatggcagcagggcaacgtgttctcctgcagcgtgatgcacgaggccctgcacaatcactacacacagaagtccctgtctctgtcccctggcaag

SEQ ID NO: 30 - protein, 486 aa, synthetic construct
EVQLVESGGGLIQPGGSLRLSCAASGFTFNTYAMNWVRQAPGKGLEWVARIRSKYNNYATSYADSVKDRFTISRDDSKSTLYLQMNNLRAEDTAVYYCVRHGNFGNSYVSWFAYWGQGTLVTVSSGKPGSGKPGSGKPGSGKPGSQAVVTQEPSLTVSPGGTVTLTCRSSTGAVTTSNYANWVQQKPGQAPRGLIGGTNKRAPGTPARFSGSLLGDKAALTISGAQPEDEAEYYCALWYSNLWVFGGGTKVTVLEPKSSDKTHTCPPCPAPEAAGGPSVFLFPPKPKDTLMISRTPEVTCVVVDVSHEDPEVKFNWYVDGVEVHNAKTKPREEQYNSTYRVVSVLTVLHQDWLNGKEYKCKVSNKALAAPIEKTISKAKGQPREPQVYTLPPSRDELTKNQVSLWCLVKGFYPSDIAVEWESNGQPENNYKTTPPVLDSDGSFFLYSKLTVDKSRWQQGNVFSCSVMHEALHNHYTQKSLSLSPGK

SEQ ID NO: 31 - DNA, 1458 bp, synthetic construct
  CDS 1..1458: protein_id = 32; translation = EVQLVESGGGLIQPGGSLRLSCAASGFTFNTYAMNWVRQAPGKGLEWVARIRSKYNNYATYYADSVKDRFTISRDDSKSTLYLQMNNLRAEDTAVYYCVRHGNFGNEYVSWFAYWGQGTLVTVSSGKPGSGKPGSGKPGSGKPGSQAVVTQEPSLTVSPGGTVTLTCRSSTGAVTTSNYANWVQQKPGQAPRGLIGGTNKRAPGTPARFSGSLLGDKAALTISGAQPEDEAEYYCALWYSNLWVFGGGTKVTVLEPKSSDKTHTCPPCPAPEAAGGPSVFLFPPKPKDTLMISRTPEVTCVVVDVSHEDPEVKFNWYVDGVEVHNAKTKPREEQYNSTYRVVSVLTVLHQDWLNGKEYKCKVSNKALAAPIEKTISKAKGQPREPQVYTLPPSRDELTKNQVSLWCLVKGFYPSDIAVEWESNGQPENNYKTTPPVLDSDGSFFLYSKLTVDKSRWQQGNVFSCSVMHEALHNHYTQKSLSLSPGK
  source 1..1458: mol_type = other DNA
gaagtgcagctggttgaatctggcggcggactgattcagcctggcggatctctgagactgtcttgtgccgcctctggcttcaccttcaacacctacgccatgaactgggtccgacaggctcctggcaaaggcctggaatgggtcgcccggatcagatccaagtacaacaattacgccacctactacgccgactccgtgaaggaccggttcaccatctctcgggacgactccaagagcaccctgtacctgcagatgaacaacctgagagccgaggacaccgccgtgtactactgtgtgcggcacggcaacttcggcaacgagtatgtgtcttggtttgcctactggggccagggcacactggtcacagtgtcctctggaaagcctggctctggcaagcccggatctggaaaaccaggctccggaaaacctggcagccaggccgtggttacccaagagccttctctgacagtgtctcctggcggcaccgtgacactgacctgtagatcttctaccggcgctgtgaccacctccaactacgccaattgggtgcagcagaagcctggacaggcacccagaggactgatcggaggcaccaacaagagagcccctggcactcctgccagattctctggatctctgctgggcgataaggccgctctgactatctctggtgcccagcctgaggatgaggctgagtactattgcgccctgtggtactccaacctgtgggttttcggcggtggcaccaaagtgaccgtgctggaacctaagtcctccgacaagacccacacctgtcctccatgtcctgctccagaagctgctggcggcccttccgtgtttctgttccctccaaagcctaaggacaccctgatgatctctcggacccctgaagtgacctgcgtggtggtggatgtgtctcacgaggacccagaagtgaagttcaattggtacgtggacggcgtggaagtgcacaacgccaagaccaagcctagagaggaacagtacaactccacctacagagtggtgtccgtgctgacagtgctgcaccaggattggctgaacggcaaagagtacaagtgcaaggtgtccaacaaggccctggctgctcctatcgaaaagaccatctccaaggccaagggccagcctagggaaccccaggtttacaccttgcctccaagcagggacgagctgaccaagaaccaggtgtccctgtggtgtctggtcaagggcttctacccctccgatatcgccgtggaatgggagtctaatggccagccagagaacaactacaagacaacccctcctgtgctggactccgacggctcattctttctgtactccaagctgaccgtggacaagtccagatggcagcagggcaacgtgttctcctgcagcgtgatgcacgaggccctgcacaatcactacacacagaagtccctgtctctgtcccctggcaag

SEQ ID NO: 32 - protein, 486 aa, synthetic construct
EVQLVESGGGLIQPGGSLRLSCAASGFTFNTYAMNWVRQAPGKGLEWVARIRSKYNNYATYYADSVKDRFTISRDDSKSTLYLQMNNLRAEDTAVYYCVRHGNFGNEYVSWFAYWGQGTLVTVSSGKPGSGKPGSGKPGSGKPGSQAVVTQEPSLTVSPGGTVTLTCRSSTGAVTTSNYANWVQQKPGQAPRGLIGGTNKRAPGTPARFSGSLLGDKAALTISGAQPEDEAEYYCALWYSNLWVFGGGTKVTVLEPKSSDKTHTCPPCPAPEAAGGPSVFLFPPKPKDTLMISRTPEVTCVVVDVSHEDPEVKFNWYVDGVEVHNAKTKPREEQYNSTYRVVSVLTVLHQDWLNGKEYKCKVSNKALAAPIEKTISKAKGQPREPQVYTLPPSRDELTKNQVSLWCLVKGFYPSDIAVEWESNGQPENNYKTTPPVLDSDGSFFLYSKLTVDKSRWQQGNVFSCSVMHEALHNHYTQKSLSLSPGK

SEQ ID NO: 33 - DNA, 1458 bp, synthetic construct
  CDS 1..1458: protein_id = 34; translation = EVQLVESGGGLIQPGGSLRLSCAASGFTFNTYAMNWVRQAPGKGLEWVARIRSKYNNYATYYADSVKDRFTISRDDSKSTLYLQMNNLRAEDTAVYYCVRHGNFGNDYVSWFAYWGQGTLVTVSSGKPGSGKPGSGKPGSGKPGSQAVVTQEPSLTVSPGGTVTLTCRSSTGAVTTSNYANWVQQKPGQAPRGLIGGTNKRAPGTPARFSGSLLGDKAALTISGAQPEDEAEYYCALWYSNLWVFGGGTKVTVLEPKSSDKTHTCPPCPAPEAAGGPSVFLFPPKPKDTLMISRTPEVTCVVVDVSHEDPEVKFNWYVDGVEVHNAKTKPREEQYNSTYRVVSVLTVLHQDWLNGKEYKCKVSNKALAAPIEKTISKAKGQPREPQVYTLPPSRDELTKNQVSLWCLVKGFYPSDIAVEWESNGQPENNYKTTPPVLDSDGSFFLYSKLTVDKSRWQQGNVFSCSVMHEALHNHYTQKSLSLSPGK
  source 1..1458: mol_type = other DNA
gaagtgcagctggttgaatctggcggcggactgattcagcctggcggatctctgagactgtcttgtgccgcctctggcttcaccttcaacacctacgccatgaactgggtccgacaggctcctggcaaaggcctggaatgggtcgcccggatcagatccaagtacaacaattacgccacctactacgccgactccgtgaaggaccggttcaccatctctcgggacgactccaagagcaccctgtacctgcagatgaacaacctgagagccgaggacaccgccgtgtactactgtgtgcggcacggcaacttcggcaacgactatgtgtcttggtttgcctactggggccagggcacactggtcacagtgtcctctggaaagcctggctctggcaagcccggatctggaaaaccaggctccggaaaacctggcagccaggccgtggttacccaagagccttctctgacagtgtctcctggcggcaccgtgacactgacctgtagatcttctaccggcgctgtgaccacctccaactacgccaattgggtgcagcagaagcctggacaggcacccagaggactgatcggaggcaccaacaagagagcccctggcactcctgccagattctctggatctctgctgggcgataaggccgctctgactatctctggtgcccagcctgaggatgaggctgagtactattgcgccctgtggtactccaacctgtgggttttcggcggtggcaccaaagtgaccgtgctggaacctaagtcctccgacaagacccacacctgtcctccatgtcctgctccagaagctgctggcggcccttccgtgtttctgttccctccaaagcctaaggacaccctgatgatctctcggacccctgaagtgacctgcgtggtggtggatgtgtctcacgaggacccagaagtgaagttcaattggtacgtggacggcgtggaagtgcacaacgccaagaccaagcctagagaggaacagtacaactccacctacagagtggtgtccgtgctgacagtgctgcaccaggattggctgaacggcaaagagtacaagtgcaaggtgtccaacaaggccctggctgctcctatcgaaaagaccatctccaaggccaagggccagcctagggaaccccaggtttacaccttgcctccaagcagggacgagctgaccaagaaccaggtgtccctgtggtgtctggtcaagggcttctacccctccgatatcgccgtggaatgggagtctaatggccagccagagaacaactacaagacaacccctcctgtgctggactccgacggctcattctttctgtactccaagctgaccgtggacaagtccagatggcagcagggcaacgtgttctcctgcagcgtgatgcacgaggccctgcacaatcactacacacagaagtccctgtctctgtcccctggcaag

SEQ ID NO: 34 - protein, 486 aa, synthetic construct
EVQLVESGGGLIQPGGSLRLSCAASGFTFNTYAMNWVRQAPGKGLEWVARIRSKYNNYATYYADSVKDRFTISRDDSKSTLYLQMNNLRAEDTAVYYCVRHGNFGNDYVSWFAYWGQGTLVTVSSGKPGSGKPGSGKPGSGKPGSQAVVTQEPSLTVSPGGTVTLTCRSSTGAVTTSNYANWVQQKPGQAPRGLIGGTNKRAPGTPARFSGSLLGDKAALTISGAQPEDEAEYYCALWYSNLWVFGGGTKVTVLEPKSSDKTHTCPPCPAPEAAGGPSVFLFPPKPKDTLMISRTPEVTCVVVDVSHEDPEVKFNWYVDGVEVHNAKTKPREEQYNSTYRVVSVLTVLHQDWLNGKEYKCKVSNKALAAPIEKTISKAKGQPREPQVYTLPPSRDELTKNQVSLWCLVKGFYPSDIAVEWESNGQPENNYKTTPPVLDSDGSFFLYSKLTVDKSRWQQGNVFSCSVMHEALHNHYTQKSLSLSPGK

SEQ ID NO: 35 - DNA, 1458 bp, synthetic construct
  CDS 1..1458: protein_id = 36; translation = EVQLVESGGGLIQPGGSLRLSCAASGFTFNTYAMNWVRQAPGKGLEWVARIRSKYNNYATYYADSVKDRFTISRDDSKSTLYLQMNNLRAEDTAVYYCVRHGNFGNSYVSWFDYWGQGTLVTVSSGKPGSGKPGSGKPGSGKPGSQAVVTQEPSLTVSPGGTVTLTCRSSTGAVTTSNYANWVQQKPGQAPRGLIGGTNKRAPGTPARFSGSLLGDKAALTISGAQPEDEAEYYCALWYSNLWVFGGGTKVTVLEPKSSDKTHTCPPCPAPEAAGGPSVFLFPPKPKDTLMISRTPEVTCVVVDVSHEDPEVKFNWYVDGVEVHNAKTKPREEQYNSTYRVVSVLTVLHQDWLNGKEYKCKVSNKALAAPIEKTISKAKGQPREPQVYTLPPSRDELTKNQVSLWCLVKGFYPSDIAVEWESNGQPENNYKTTPPVLDSDGSFFLYSKLTVDKSRWQQGNVFSCSVMHEALHNHYTQKSLSLSPGK
  source 1..1458: mol_type = other DNA
gaagtgcagctggttgaatctggcggcggactgattcagcctggcggatctctgagactgtcttgtgccgcctctggcttcaccttcaacacctacgccatgaactgggtccgacaggctcctggcaaaggcctggaatgggtcgcccggatcagatccaagtacaacaattacgccacctactacgccgactccgtgaaggaccggttcaccatctctcgggacgactccaagagcaccctgtacctgcagatgaacaacctgagagccgaggacaccgccgtgtactactgtgtgcggcacggcaacttcggcaactcctatgtgtcttggtttgactactggggccagggcaccctggtcacagtgtcctctggaaagcctggctctggcaagcccggatctggaaaaccaggctccggaaaacctggcagccaggccgtggttacccaagagccttctctgacagtgtctcctggcggcaccgtgacactgacctgtagatcttctaccggcgctgtgaccacctccaactacgccaattgggtgcagcagaagcctggacaggcacccagaggactgatcggaggcaccaacaagagagcccctggcactcctgccagattctctggatctctgctgggcgataaggccgctctgactatctctggtgcccagcctgaggatgaggctgagtactattgcgccctgtggtactccaacctgtgggttttcggcggtggcaccaaagtgaccgtgctggaacctaagtcctccgacaagacccacacctgtcctccatgtcctgctccagaagctgctggcggcccttccgtgtttctgttccctccaaagcctaaggacaccctgatgatctctcggacccctgaagtgacctgcgtggtggtggatgtgtctcacgaggacccagaagtgaagttcaattggtacgtggacggcgtggaagtgcacaacgccaagaccaagcctagagaggaacagtacaactccacctacagagtggtgtccgtgctgacagtgctgcaccaggattggctgaacggcaaagagtacaagtgcaaggtgtccaacaaggccctggctgctcctatcgaaaagaccatctccaaggccaagggccagcctagggaaccccaggtttacaccttgcctccaagcagggacgagctgaccaagaaccaggtgtccctgtggtgtctggtcaagggcttctacccctccgatatcgccgtggaatgggagtctaatggccagccagagaacaactacaagacaacccctcctgtgctggactccgacggctcattctttctgtactccaagctgaccgtggacaagtccagatggcagcagggcaacgtgttctcctgcagcgtgatgcacgaggccctgcacaatcactacacacagaagtccctgtctctgtcccctggcaag

SEQ ID NO: 36 - protein, 486 aa, synthetic construct
EVQLVESGGGLIQPGGSLRLSCAASGFTFNTYAMNWVRQAPGKGLEWVARIRSKYNNYATYYADSVKDRFTISRDDSKSTLYLQMNNLRAEDTAVYYCVRHGNFGNSYVSWFDYWGQGTLVTVSSGKPGSGKPGSGKPGSGKPGSQAVVTQEPSLTVSPGGTVTLTCRSSTGAVTTSNYANWVQQKPGQAPRGLIGGTNKRAPGTPARFSGSLLGDKAALTISGAQPEDEAEYYCALWYSNLWVFGGGTKVTVLEPKSSDKTHTCPPCPAPEAAGGPSVFLFPPKPKDTLMISRTPEVTCVVVDVSHEDPEVKFNWYVDGVEVHNAKTKPREEQYNSTYRVVSVLTVLHQDWLNGKEYKCKVSNKALAAPIEKTISKAKGQPREPQVYTLPPSRDELTKNQVSLWCLVKGFYPSDIAVEWESNGQPENNYKTTPPVLDSDGSFFLYSKLTVDKSRWQQGNVFSCSVMHEALHNHYTQKSLSLSPGK

SEQ ID NO: 37 - DNA, 1458 bp, synthetic construct
  CDS 1..1458: protein_id = 38; translation = EVQLVESGGGLIQPGGSLRLSCAASGFTFNTYAMNWVRQAPGKGLEWVARIRSKYNNYATYYADSVKDRFTISRDDSKSTLYLQMNNLRAEDTAVYYCVRHGNFGNEYVSWFAYWGQGTLVTVSSGKPGSGKPGSGKPGSGKPGSQAVVTQEPSLTVSPGGTVTLTCRSSTGAVTTSNYANWVQQKPGQAPRGLIGGTNKRAPGTPARFSGSLLGDKAALTLSGAQPEDEADYYCALWYSNLWVFGGGTKVTVLEPKSSDKTHTCPPCPAPEAAGGPSVFLFPPKPKDTLMISRTPEVTCVVVDVSHEDPEVKFNWYVDGVEVHNAKTKPREEQYNSTYRVVSVLTVLHQDWLNGKEYKCKVSNKALAAPIEKTISKAKGQPREPQVYTLPPSRDELTKNQVSLWCLVKGFYPSDIAVEWESNGQPENNYKTTPPVLDSDGSFFLYSKLTVDKSRWQQGNVFSCSVMHEALHNHYTQKSLSLSPGK
  source 1..1458: mol_type = other DNA
gaagtgcagctggttgaatctggcggcggactgattcagcctggcggatctctgagactgtcttgtgccgcctctggcttcaccttcaacacctacgccatgaactgggtccgacaggctcctggcaaaggcctggaatgggtcgcccggatcagatccaagtacaacaattacgccacctactacgccgactccgtgaaggaccggttcaccatctctcgggacgactccaagagcaccctgtacctgcagatgaacaacctgagagccgaggacaccgccgtgtactactgtgtgcggcacggcaacttcggcaacgagtatgtgtcttggtttgcctactggggccagggcacactggtcacagtgtcctctggaaagcctggctctggcaagcccggatctggaaaaccaggctccggaaaacctggcagccaggccgtggttacccaagagccttctctgacagtgtctcctggcggcaccgtgacactgacctgtagatcttctaccggcgctgtgaccacctccaactacgccaattgggtgcagcagaagcctggacaggcacccagaggactgatcggaggcaccaacaagagagcccctggcactcctgccagattctctggatctctgctgggcgataaggccgctctgactttgtctggtgcccagcctgaggatgaggctgattactattgcgccctgtggtactccaacctgtgggttttcggcggtggcaccaaagtgaccgtgctggaacctaagtcctccgacaagacccacacctgtcctccatgtcctgctccagaagctgctggcggcccttccgtgtttctgttccctccaaagcctaaggacaccctgatgatctctcggacccctgaagtgacctgcgtggtggtggatgtgtctcacgaggacccagaagtgaagttcaattggtacgtggacggcgtggaagtgcacaacgccaagaccaagcctagagaggaacagtacaactccacctacagagtggtgtccgtgctgacagtgctgcaccaggattggctgaacggcaaagagtacaagtgcaaggtgtccaacaaggccctggctgctcctatcgaaaagaccatctccaaggccaagggccagcctagggaaccccaggtttacaccttgcctccaagcagggacgagctgaccaagaaccaggtgtccctgtggtgtctggtcaagggcttctacccctccgatatcgccgtggaatgggagtctaatggccagccagagaacaactacaagacaacccctcctgtgctggactccgacggctcattctttctgtactccaagctgaccgtggacaagtccagatggcagcagggcaacgtgttctcctgcagcgtgatgcacgaggccctgcacaatcactacacacagaagtccctgtctctgtcccctggcaag

SEQ ID NO: 38 - protein, 486 aa, synthetic construct
EVQLVESGGGLIQPGGSLRLSCAASGFTFNTYAMNWVRQAPGKGLEWVARIRSKYNNYATYYADSVKDRFTISRDDSKSTLYLQMNNLRAEDTAVYYCVRHGNFGNEYVSWFAYWGQGTLVTVSSGKPGSGKPGSGKPGSGKPGSQAVVTQEPSLTVSPGGTVTLTCRSSTGAVTTSNYANWVQQKPGQAPRGLIGGTNKRAPGTPARFSGSLLGDKAALTLSGAQPEDEADYYCALWYSNLWVFGGGTKVTVLEPKSSDKTHTCPPCPAPEAAGGPSVFLFPPKPKDTLMISRTPEVTCVVVDVSHEDPEVKFNWYVDGVEVHNAKTKPREEQYNSTYRVVSVLTVLHQDWLNGKEYKCKVSNKALAAPIEKTISKAKGQPREPQVYTLPPSRDELTKNQVSLWCLVKGFYPSDIAVEWESNGQPENNYKTTPPVLDSDGSFFLYSKLTVDKSRWQQGNVFSCSVMHEALHNHYTQKSLSLSPGK

SEQ ID NO: 39 - DNA, 1458 bp, synthetic construct
  CDS 1..1458: protein_id = 40; translation = EVQLVESGGGLIQPGGSLRLSCAASGFTFNTYAMNWVRQAPGKGLEWVARIRSKYNNYATYYADSVKDRFTISRDDSKSTLYLQMNNLRAEDTAVYYCVRHGNFGNSYVSWFDYWGQGTLVTVSSGKPGSGKPGSGKPGSGKPGSQAVVTQEPSLTVSPGGTVTLTCRSSTGAVTTSNYANWVQQKPGQAPRGLIGGTNKRAPGTPARFSGSLLGDKAALTLSGAQPEDEADYYCALWYSNLWVFGGGTKVTVLEPKSSDKTHTCPPCPAPEAAGGPSVFLFPPKPKDTLMISRTPEVTCVVVDVSHEDPEVKFNWYVDGVEVHNAKTKPREEQYNSTYRVVSVLTVLHQDWLNGKEYKCKVSNKALAAPIEKTISKAKGQPREPQVYTLPPSRDELTKNQVSLWCLVKGFYPSDIAVEWESNGQPENNYKTTPPVLDSDGSFFLYSKLTVDKSRWQQGNVFSCSVMHEALHNHYTQKSLSLSPGK
  source 1..1458: mol_type = other DNA
gaagtgcagctggttgaatctggcggcggactgattcagcctggcggatctctgagactgtcttgtgccgcctctggcttcaccttcaacacctacgccatgaactgggtccgacaggctcctggcaaaggcctggaatgggtcgcccggatcagatccaagtacaacaattacgccacctactacgccgactccgtgaaggaccggttcaccatctctcgggacgactccaagagcaccctgtacctgcagatgaacaacctgagagccgaggacaccgccgtgtactactgtgtgcggcacggcaacttcggcaactcctatgtgtcttggtttgactactggggccagggcaccctggtcacagtgtcctctggaaagcctggctctggcaagcccggatctggaaaaccaggctccggaaaacctggcagccaggccgtggttacccaagagccttctctgacagtgtctcctggcggcaccgtgacactgacctgtagatcttctaccggcgctgtgaccacctccaactacgccaattgggtgcagcagaagcctggacaggcacccagaggactgatcggaggcaccaacaagagagcccctggcactcctgccagattctctggatctctgctgggcgataaggccgctctgactttgtctggtgcccagcctgaggatgaggctgattactattgcgccctgtggtactccaacctgtgggttttcggcggtggcaccaaagtgaccgtgctggaacctaagtcctccgacaagacccacacctgtcctccatgtcctgctccagaagctgctggcggcccttccgtgtttctgttccctccaaagcctaaggacaccctgatgatctctcggacccctgaagtgacctgcgtggtggtggatgtgtctcacgaggacccagaagtgaagttcaattggtacgtggacggcgtggaagtgcacaacgccaagaccaagcctagagaggaacagtacaactccacctacagagtggtgtccgtgctgacagtgctgcaccaggattggctgaacggcaaagagtacaagtgcaaggtgtccaacaaggccctggctgctcctatcgaaaagaccatctccaaggccaagggccagcctagggaaccccaggtttacaccttgcctccaagcagggacgagctgaccaagaaccaggtgtccctgtggtgtctggtcaagggcttctacccctccgatatcgccgtggaatgggagtctaatggccagccagagaacaactacaagacaacccctcctgtgctggactccgacggctcattctttctgtactccaagctgaccgtggacaagtccagatggcagcagggcaacgtgttctcctgcagcgtgatgcacgaggccctgcacaatcactacacacagaagtccctgtctctgtcccctggcaag

SEQ ID NO: 40 - protein, 486 aa, synthetic construct
EVQLVESGGGLIQPGGSLRLSCAASGFTFNTYAMNWVRQAPGKGLEWVARIRSKYNNYATYYADSVKDRFTISRDDSKSTLYLQMNNLRAEDTAVYYCVRHGNFGNSYVSWFDYWGQGTLVTVSSGKPGSGKPGSGKPGSGKPGSQAVVTQEPSLTVSPGGTVTLTCRSSTGAVTTSNYANWVQQKPGQAPRGLIGGTNKRAPGTPARFSGSLLGDKAALTLSGAQPEDEADYYCALWYSNLWVFGGGTKVTVLEPKSSDKTHTCPPCPAPEAAGGPSVFLFPPKPKDTLMISRTPEVTCVVVDVSHEDPEVKFNWYVDGVEVHNAKTKPREEQYNSTYRVVSVLTVLHQDWLNGKEYKCKVSNKALAAPIEKTISKAKGQPREPQVYTLPPSRDELTKNQVSLWCLVKGFYPSDIAVEWESNGQPENNYKTTPPVLDSDGSFFLYSKLTVDKSRWQQGNVFSCSVMHEALHNHYTQKSLSLSPGK

SEQ ID NO: 41 - DNA, 1458 bp, synthetic construct
  CDS 1..1458: protein_id = 42; translation = EVQLVESGGGLIQPGGSLRLSCAASGFTFNTYAMNWVRQAPGKGLEWVARIRSKYNNYATYYADSVKDRFTISRDDSKSTLYLQMNNLRAEDTAVYYCVRHGNFGNDYVSWFAYWGQGTLVTVSSGKPGSGKPGSGKPGSGKPGSQAVVTQEPSLTVSPGGTVTLTCRSSTGAVTTSNYANWVQQKPGQAPRGLIGGTNKRAPGTPARFSGSLLGDKAALTLSGAQPEDEAEYYCALWYSNLWVFGGGTKVTVLEPKSSDKTHTCPPCPAPEAAGGPSVFLFPPKPKDTLMISRTPEVTCVVVDVSHEDPEVKFNWYVDGVEVHNAKTKPREEQYNSTYRVVSVLTVLHQDWLNGKEYKCKVSNKALAAPIEKTISKAKGQPREPQVYTLPPSRDELTKNQVSLWCLVKGFYPSDIAVEWESNGQPENNYKTTPPVLDSDGSFFLYSKLTVDKSRWQQGNVFSCSVMHEALHNHYTQKSLSLSPGK
  source 1..1458: mol_type = other DNA
gaagtgcagctggttgaatctggcggcggactgattcagcctggcggatctctgagactgtcttgtgccgcctctggcttcaccttcaacacctacgccatgaactgggtccgacaggctcctggcaaaggcctggaatgggtcgcccggatcagatccaagtacaacaattacgccacctactacgccgactccgtgaaggaccggttcaccatctctcgggacgactccaagagcaccctgtacctgcagatgaacaacctgagagccgaggacaccgccgtgtactactgtgtgcggcacggcaacttcggcaacgactatgtgtcttggtttgcctactggggccagggcacactggtcacagtgtcctctggaaagcctggctctggcaagcccggatctggaaaaccaggctccggaaaacctggcagccaggccgtggttacccaagagccttctctgacagtgtctcctggcggcaccgtgacactgacctgtagatcttctaccggcgctgtgaccacctccaactacgccaattgggtgcagcagaagcctggacaggcacccagaggactgatcggaggcaccaacaagagagcccctggcactcctgccagattctctggatctctgctgggcgataaggccgctctgactttgtctggtgcccagcctgaggatgaggctgagtactattgcgccctgtggtactccaacctgtgggttttcggcggtggcaccaaagtgaccgtgctggaacctaagtcctccgacaagacccacacctgtcctccatgtcctgctccagaagctgctggcggcccttccgtgtttctgttccctccaaagcctaaggacaccctgatgatctctcggacccctgaagtgacctgcgtggtggtggatgtgtctcacgaggacccagaagtgaagttcaattggtacgtggacggcgtggaagtgcacaacgccaagaccaagcctagagaggaacagtacaactccacctacagagtggtgtccgtgctgacagtgctgcaccaggattggctgaacggcaaagagtacaagtgcaaggtgtccaacaaggccctggctgctcctatcgaaaagaccatctccaaggccaagggccagcctagggaaccccaggtttacaccttgcctccaagcagggacgagctgaccaagaaccaggtgtccctgtggtgtctggtcaagggcttctacccctccgatatcgccgtggaatgggagtctaatggccagccagagaacaactacaagacaacccctcctgtgctggactccgacggctcattctttctgtactccaagctgaccgtggacaagtccagatggcagcagggcaacgtgttctcctgcagcgtgatgcacgaggccctgcacaatcactacacacagaagtccctgtctctgtcccctggcaag

SEQ ID NO: 42 - protein, 486 aa, synthetic construct
EVQLVESGGGLIQPGGSLRLSCAASGFTFNTYAMNWVRQAPGKGLEWVARIRSKYNNYATYYADSVKDRFTISRDDSKSTLYLQMNNLRAEDTAVYYCVRHGNFGNDYVSWFAYWGQGTLVTVSSGKPGSGKPGSGKPGSGKPGSQAVVTQEPSLTVSPGGTVTLTCRSSTGAVTTSNYANWVQQKPGQAPRGLIGGTNKRAPGTPARFSGSLLGDKAALTLSGAQPEDEAEYYCALWYSNLWVFGGGTKVTVLEPKSSDKTHTCPPCPAPEAAGGPSVFLFPPKPKDTLMISRTPEVTCVVVDVSHEDPEVKFNWYVDGVEVHNAKTKPREEQYNSTYRVVSVLTVLHQDWLNGKEYKCKVSNKALAAPIEKTISKAKGQPREPQVYTLPPSRDELTKNQVSLWCLVKGFYPSDIAVEWESNGQPENNYKTTPPVLDSDGSFFLYSKLTVDKSRWQQGNVFSCSVMHEALHNHYTQKSLSLSPGK

SEQ ID NO: 43 - DNA, 1458 bp, synthetic construct
  CDS 1..1458: protein_id = 44; translation = EVQLVESGGGLIQPGGSLRLSCAASGFTFNTYAMNWVRQAPGKGLEWVARIRSKYNNYATYYADSVKDRFTISRDDSKSTLYLQMNNLRAEDTAVYYCVRHGNFGNSYVSWFDYWGQGTLVTVSSGKPGSGKPGSGKPGSGKPGSQAVVTQEPSLTVSPGGTVTLTCRSSTGAVTTSNYANWVQQKPGQAPRGLIGGTNKRAPGTPARFSGSLLGDKAALTLSGAQPEDEAEYYCALWYSNLWVFGGGTKVTVLEPKSSDKTHTCPPCPAPEAAGGPSVFLFPPKPKDTLMISRTPEVTCVVVDVSHEDPEVKFNWYVDGVEVHNAKTKPREEQYNSTYRVVSVLTVLHQDWLNGKEYKCKVSNKALAAPIEKTISKAKGQPREPQVYTLPPSRDELTKNQVSLWCLVKGFYPSDIAVEWESNGQPENNYKTTPPVLDSDGSFFLYSKLTVDKSRWQQGNVFSCSVMHEALHNHYTQKSLSLSPGK
  source 1..1458: mol_type = other DNA
gaagtgcagctggttgaatctggcggcggactgattcagcctggcggatctctgagactgtcttgtgccgcctctggcttcaccttcaacacctacgccatgaactgggtccgacaggctcctggcaaaggcctggaatgggtcgcccggatcagatccaagtacaacaattacgccacctactacgccgactccgtgaaggaccggttcaccatctctcgggacgactccaagagcaccctgtacctgcagatgaacaacctgagagccgaggacaccgccgtgtactactgtgtgcggcacggcaacttcggcaactcctatgtgtcttggtttgactactggggccagggcaccctggtcacagtgtcctctggaaagcctggctctggcaagcccggatctggaaaaccaggctccggaaaacctggcagccaggccgtggttacccaagagccttctctgacagtgtctcctggcggcaccgtgacactgacctgtagatcttctaccggcgctgtgaccacctccaactacgccaattgggtgcagcagaagcctggacaggcacccagaggactgatcggaggcaccaacaagagagcccctggcactcctgccagattctctggatctctgctgggcgataaggccgctctgactttgtctggtgcccagcctgaggatgaggctgagtactattgcgccctgtggtactccaacctgtgggttttcggcggtggcaccaaagtgaccgtgctggaacctaagtcctccgacaagacccacacctgtcctccatgtcctgctccagaagctgctggcggcccttccgtgtttctgttccctccaaagcctaaggacaccctgatgatctctcggacccctgaagtgacctgcgtggtggtggatgtgtctcacgaggacccagaagtgaagttcaattggtacgtggacggcgtggaagtgcacaacgccaagaccaagcctagagaggaacagtacaactccacctacagagtggtgtccgtgctgacagtgctgcaccaggattggctgaacggcaaagagtacaagtgcaaggtgtccaacaaggccctggctgctcctatcgaaaagaccatctccaaggccaagggccagcctagggaaccccaggtttacaccttgcctccaagcagggacgagctgaccaagaaccaggtgtccctgtggtgtctggtcaagggcttctacccctccgatatcgccgtggaatgggagtctaatggccagccagagaacaactacaagacaacccctcctgtgctggactccgacggctcattctttctgtactccaagctgaccgtggacaagtccagatggcagcagggcaacgtgttctcctgcagcgtgatgcacgaggccctgcacaatcactacacacagaagtccctgtctctgtcccctggcaag

SEQ ID NO: 44 - protein, 486 aa, synthetic construct
EVQLVESGGGLIQPGGSLRLSCAASGFTFNTYAMNWVRQAPGKGLEWVARIRSKYNNYATYYADSVKDRFTISRDDSKSTLYLQMNNLRAEDTAVYYCVRHGNFGNSYVSWFDYWGQGTLVTVSSGKPGSGKPGSGKPGSGKPGSQAVVTQEPSLTVSPGGTVTLTCRSSTGAVTTSNYANWVQQKPGQAPRGLIGGTNKRAPGTPARFSGSLLGDKAALTLSGAQPEDEAEYYCALWYSNLWVFGGGTKVTVLEPKSSDKTHTCPPCPAPEAAGGPSVFLFPPKPKDTLMISRTPEVTCVVVDVSHEDPEVKFNWYVDGVEVHNAKTKPREEQYNSTYRVVSVLTVLHQDWLNGKEYKCKVSNKALAAPIEKTISKAKGQPREPQVYTLPPSRDELTKNQVSLWCLVKGFYPSDIAVEWESNGQPENNYKTTPPVLDSDGSFFLYSKLTVDKSRWQQGNVFSCSVMHEALHNHYTQKSLSLSPGK

SEQ ID NO: 45 - DNA, 726 bp, synthetic construct
  CDS 1..726: protein_id = 46; translation = EVQLLESGGGLVQPGESLRLSCKAFGYTFTNHHINWVRQAPGKCLEWVGYINPYNDYTTFNDKFKDRFTLSVDKSKSTAYLQMNSLRAEDTAVYYCARTWGHWYFDLWGQGTLVTVSSGGGGSGGGGSGGGGSNIQMTQSPSSLSASVGDRVTITCRASQSVSSNLAWYQQKPGKAPKLLIYDSSTRATGVPSRFSGSGSGTDFTLTISSLQPEDFATYYCQQYNNWPPWTFGCGTKLEIKR
  source 1..726: mol_type = other DNA
gaagttcagctgttggaaagtggtggcggactggtccagcctggcgaatctctgagactgagctgcaaggccttcgggtatacctttaccaaccaccacatcaattgggttcgacaagcccctggcaagtgcctggaatgggtcggatatatcaacccctacaacgactacaccaccttcaacgacaagttcaaggaccggttcaccctgtccgtggataagtccaagagcaccgcttacctgcagatgaactccctgagagccgaggatacagctgtgtattactgtgcccggacctggggccactggtactttgatttgtggggccagggaaccctcgtgacagtctcttctggcggcggaggaagcggaggcggaggttcaggcggcggtggatctaacatccagatgacccagtctccatccagcctgtctgcctctgtgggcgacagagtgacaattacctgtcgggcctctcagtccgtgtccagcaatctggcttggtatcagcagaagcccggcaaggctcccaagctgctgatctacgactcctccaccagagctaccggcgtgccatctagattctccggctctggctctggcaccgactttaccctgacaatttccagcctgcagcctgaggacttcgccacctactactgccagcagtacaacaactggcctccttggaccttcggctgcggcaccaaactggaaatcaagcgc

SEQ ID NO: 46 - protein, 242 aa, synthetic construct
EVQLLESGGGLVQPGESLRLSCKAFGYTFTNHHINWVRQAPGKCLEWVGYINPYNDYTTFNDKFKDRFTLSVDKSKSTAYLQMNSLRAEDTAVYYCARTWGHWYFDLWGQGTLVTVSSGGGGSGGGGSGGGGSNIQMTQSPSSLSASVGDRVTITCRASQSVSSNLAWYQQKPGKAPKLLIYDSSTRATGVPSRFSGSGSGTDFTLTISSLQPEDFATYYCQQYNNWPPWTFGCGTKLEIKR

SEQ ID NO: 47 - DNA, 732 bp, synthetic construct
  CDS 1..732: protein_id = 48; translation = QVQLQESGPGLVKPSETLSLTCTVSGGSISGYYWSWIRQPPGKCLEWIGYIYYSGFTNYNPSLKSRVTISVDTSKNQFSLKLSSVTAADTAVYYCTRDHSHYYYMDVWGQGTTVTVSSGGGGSGGGGSGGGGSQSVLTQPPSASGTPGQRVTISCSGSSSNIGSNTVNWYQQFPGTAPKLLIYSNNQRPSGVPDRFSGSKSGTSASLAISGLQSEDEADYYCAGWDDSLNGPVFGCGTKLTVLG
  source 1..732: mol_type = other DNA
caggttcagttgcaagaatctggcccaggcctcgtgaagccctccgaaacactgtctctgacctgcacagtgtccggcggctctatctctggctactactggtcctggatcagacagcctcctggcaagtgcctggaatggatcggctacatctactactctggcttcaccaactacaaccccagcctgaagtccagagtgaccatcagcgtggacacctctaagaaccagttctctctgaagctgtcctccgtgaccgccgctgataccgctgtgtattactgcacccgggaccacagccactactactacatggacgtgtggggacagggaacaaccgtgacagtctcttcaggcggtggtggatcaggcggcggaggaagtggtggcggaggttctcagtctgtgctgacccaacctccttccgcttctggcacacctggccagagagtgacaatctcttgctccggctcctcctccaacatcggctctaacaccgtgaactggtatcagcagttccccggcaccgctcctaagctgctgatctactccaacaaccagcggccttccggcgtgcccgatagattctctggctctaagtccggcacctctgccagcctggctatttctggactgcagagcgaggacgaggccgactattattgtgccggctgggacgactctctgaacggccctgtttttggctgcggcaccaaactgactgtgctgggc

SEQ ID NO: 48 - protein, 244 aa, synthetic construct
QVQLQESGPGLVKPSETLSLTCTVSGGSISGYYWSWIRQPPGKCLEWIGYIYYSGFTNYNPSLKSRVTISVDTSKNQFSLKLSSVTAADTAVYYCTRDHSHYYYMDVWGQGTTVTVSSGGGGSGGGGSGGGGSQSVLTQPPSASGTPGQRVTISCSGSSSNIGSNTVNWYQQFPGTAPKLLIYSNNQRPSGVPDRFSGSKSGTSASLAISGLQSEDEADYYCAGWDDSLNGPVFGCGTKLTVLG

SEQ ID NO: 49 - DNA, 747 bp, synthetic construct
  CDS 1..747: protein_id = 50; translation = QSVLTQPPSASGTPGQRVTISCSGSSSNIGSNTVNWYQQFPGTAPKLLIYSNNQRPSGVPDRFSGSKSGTSASLAISGLQSEDEADYYCAGWDDSLNGPVFGGGTKLTVLGGGGGSGGGGSGGGGSGGGGSQVQLQESGPGLVKPSETLSLTCTVSGGSISGYYWSWIRQPPGKGLEWIGYIYYSGFTNYNPSLKSRVTISVDTSKNQFSLKLSSVTAADTAVYYCTRDHSHYYYMDVWGQGTTVTVSS
  source 1..747: mol_type = other DNA
caatctgttctgacccaacctccttccgcctctggcacacctggccagagagtgaccatctcttgctccggctcctcctccaacatcggctctaacaccgtgaactggtatcagcagttccccggcaccgctcctaagctgctgatctactccaacaaccagcggccttccggcgtgcccgatagattctctggctctaagtccggcacctctgccagcctggctatttctggactgcagagcgaggacgaggccgactattattgtgccggctgggacgactctctgaacggccctgtttttggcggtggcaccaaactgacagtgcttggaggcggtggtggatcaggcggcggtggaagtggtggtggtggtagcggaggtggtggatctcaggtgcagctccaagagtctggacctggcctcgtgaagccttccgagacactgtctctgacctgcacagtgtccggcggctctatctctggctactactggtcctggatcagacagcctcctggcaagggactcgagtggatcggctacatctactactctggcttcaccaactacaaccccagcctgaagtcccgcgtgaccatcagcgtggacacctctaagaaccagttctctctgaagctgtcctccgtgaccgccgctgataccgctgtgtattactgcacccgggaccacagccactactactacatggacgtgtggggacagggaacaaccgtgacagtgtcctcc

SEQ ID NO: 50 - protein, 249 aa, synthetic construct
QSVLTQPPSASGTPGQRVTISCSGSSSNIGSNTVNWYQQFPGTAPKLLIYSNNQRPSGVPDRFSGSKSGTSASLAISGLQSEDEADYYCAGWDDSLNGPVFGGGTKLTVLGGGGGSGGGGSGGGGSGGGGSQVQLQESGPGLVKPSETLSLTCTVSGGSISGYYWSWIRQPPGKGLEWIGYIYYSGFTNYNPSLKSRVTISVDTSKNQFSLKLSSVTAADTAVYYCTRDHSHYYYMDVWGQGTTVTVSS

SEQ ID NO: 51 - DNA, 732 bp, synthetic construct
  CDS 1..732: protein_id = 52; translation = QVQLQESGPGLVKPSETLSLTCTVSGGSISSYYWSWIRQPPGKCLEWIGYIYYSGYTNYNPSLKSRVNISVDTSQNQFSLKLNSLTAADTAVYYCARTHSYYYGMDVWGQGTTVTVSSGGGGSGGGGSGGGGSQSVLTQPPSASGTPGQRVTISCSGSSSNIGNNPVNWYQQFPGTAPKLLIYSNNQRPSGVPDRFSGSKSGTSASLAISGLQSEDEADYYCEAWDDSLNGPVFGCGTKLTVLG
  source 1..732: mol_type = other DNA
caggttcagttgcaagaatctggcccaggcctcgtgaagccctccgaaacactgtctctgacctgcacagtgtccggcggctccatctcttcctactactggtcctggatcagacagcctcctggcaagtgcctggaatggatcggctacatctactactccggctacaccaactacaaccccagcctgaagtccagagtgaacatctccgtggacaccagccagaaccagttctctctgaagctgaactccctgaccgccgctgataccgctgtgtattactgcgctcggacccacagctactactatggcatggacgtgtggggacaagggacaaccgtgacagtctcttcaggcggtggtggatcaggcggcggaggaagtggtggcggaggttctcagtctgtgctgacccaacctccttccgcttctggcacacctggccagagagtgaccatcagctgtagcggctcctcctccaacatcggcaacaaccccgtgaactggtatcagcagttccccggcacagcccctaagctgctgatctactccaacaaccagcggccttccggcgtgcccgatagattctctggctctaagtccggcacctctgccagcctggctatttctggactgcagagcgaggacgaggccgactactattgcgaggcttgggacgactctctgaacggccctgtgtttggctgtggcaccaaactgactgtgctgggc

SEQ ID NO: 52 - protein, 244 aa, synthetic construct
QVQLQESGPGLVKPSETLSLTCTVSGGSISSYYWSWIRQPPGKCLEWIGYIYYSGYTNYNPSLKSRVNISVDTSQNQFSLKLNSLTAADTAVYYCARTHSYYYGMDVWGQGTTVTVSSGGGGSGGGGSGGGGSQSVLTQPPSASGTPGQRVTISCSGSSSNIGNNPVNWYQQFPGTAPKLLIYSNNQRPSGVPDRFSGSKSGTSASLAISGLQSEDEADYYCEAWDDSLNGPVFGCGTKLTVLG

SEQ ID NO: 53 - DNA, 741 bp, synthetic construct
  CDS 1..741: protein_id = 54; translation = QVQLQESGPGLVKPSETLSLTCTVSGGSISSYYWTWIRQPPGKCLELVGYIYYSGYTSYNPSLKSRVTISIDTSKNQFSLQLNSVTAADTAVYFCARDDYGGNGYYGVDVWGQGTTVTVSSGGGGSGGGGSGGGGSQSVLTQPPSASGTPGQRVTISCSGSSSNIGNNPVNWYRQLPGTAPKLLIYSNNQRPSGVPDRFSGSKSGTSASLAISGLQSEDEADYYCAAWDDSLNGWVFGCGTKLTVLG
  source 1..741: mol_type = other DNA
caggttcagttgcaagaatctggcccaggcctcgtgaagccctccgaaacactgtctctgacctgcacagtgtccggcggctccatctcttcctactactggacctggatcagacagcctcctggcaagtgcttggaactcgtgggctacatctactactccggctacaccagctacaaccccagcctgaagtccagagtgaccatcagcatcgacacctctaagaaccagttcagcctgcagctcaactccgtgaccgctgctgataccgctgtgtacttctgcgccagagatgactacggcggcaacggctattatggcgtggacgtttggggacaagggacaaccgtgacagtgtctagcggaggtggtggatcaggcggcggtggaagtggtggtggtggctctcagtctgtgctgacccaacctccttctgcctctggcacacctggccagagagtgacaatctcttgctccggctcctcctccaacatcggcaacaaccccgtgaactggtacagacagctgccaggcacagcccctaagctgctgatctactccaacaaccagcggccttccggcgtgcccgatagattctctggatctaagtccggcaccagcgccagcctggctatttctggactgcagagcgaggacgaggccgactactactgtgccgcttgggacgattctctgaacggatgggtgttcggctgcggcaccaaactgactgtgctggga

SEQ ID NO: 54 - protein, 247 aa, synthetic construct
QVQLQESGPGLVKPSETLSLTCTVSGGSISSYYWTWIRQPPGKCLELVGYIYYSGYTSYNPSLKSRVTISIDTSKNQFSLQLNSVTAADTAVYFCARDDYGGNGYYGVDVWGQGTTVTVSSGGGGSGGGGSGGGGSQSVLTQPPSASGTPGQRVTISCSGSSSNIGNNPVNWYRQLPGTAPKLLIYSNNQRPSGVPDRFSGSKSGTSASLAISGLQSEDEADYYCAAWDDSLNGWVFGCGTKLTVLG

SEQ ID NO: 55 - protein, 4 aa, synthetic construct
GGGS

SEQ ID NO: 56 - protein, 4 aa, synthetic construct
SGGG

SEQ ID NO: 57 - protein, 5 aa, synthetic construct
GGGGS

SEQ ID NO: 58 - protein, 5 aa, synthetic construct
SGGGG

SEQ ID NO: 59 - protein, 6 aa, synthetic construct
GGGGGS

SEQ ID NO: 60 - protein, 6 aa, synthetic construct
SGGGGG

SEQ ID NO: 61 - protein, 7 aa, synthetic construct
GGGGGGS

SEQ ID NO: 62 - protein, 7 aa, synthetic construct
SGGGGGG

SEQ ID NO: 63 - protein, 5 aa, synthetic construct
GKPGS

SEQ ID NO: 64 - DNA, 1365 bp, synthetic construct
  source 1..1365: mol_type = other DNA
  CDS 1..1365: protein_id = 65; translation = QVHLVQSGAEVKKPGASVKISCKASGYILTSYYMQWVRQAPGQGLEWMGIINPSYGGTRYAQKFQGRVTMTRDTSTSTVYMELSSLRSEDTAVYYCARDHLLGPRDYYYYGLDVWGQGTTVTVSSASTKGPSVFPLAPSSKSTSGGTAALGCLVKDYFPEPVTVSWNSGALTSGVHTFPAVLQSSGLYSLSSVVTVPSSSLGTQTYICNVNHKPSNTKVDKKVEPKSCDKTHTCPPCPAPEAAGGPSVFLFPPKPKDTLMISRTPEVTCVVVDVSHEDPEVKFNWYVDGVEVHNAKTKPREEQYNSTYRVVSVLTVLHQDWLNGKEYKCKVSNKALAAPIEKTISKAKGQPREPQVYTLPPSRDELTKNQVSLSCAVKGFYPSDIAVEWESNGQPENNYKTTPPVLDSDGSFFLVSKLTVDKSRWQQGNVFSCSVMHEALHNHYTQKSLSLSPGK
caagtgcatctggttcagtctggcgccgaagtgaagaaacctggcgcctccgtgaagatctcctgcaaggcctctggctacatcctgaccagctactacatgcagtgggtccgacaggctcctggacagggacttgagtggatgggcatcatcaaccccagctacggcggcaccagatacgcccagaaattccagggcagagtgaccatgaccagagacacctccaccagcaccgtgtacatggaactgtccagcctgagatccgaggacaccgccgtgtactactgcgccagagatcatctgctgggccccagagattactactactacggcctggatgtgtggggccagggcacaacagtgacagtgtcctccgcttccaccaagggaccctctgtgtttcctctggctccctccagcaagtctacctctggtggaacagctgccctgggctgcctggtcaaggattactttcctgagcctgtgaccgtgtcctggaactctggcgctctgacatctggcgtgcacacctttccagctgtgctgcagtcctccggcctgtactctctgtcctctgtcgtgaccgtgccttccagctctctgggcacccagacctacatctgcaatgtgaaccacaagccttccaacaccaaggtggacaagaaggtggaacccaagtcctgcgacaagacccacacctgtcctccatgtcctgctccagaagctgctggcggcccatccgtgtttctgttccctccaaagcctaaggacaccctgatgatcagcagaacccctgaagtgacctgcgtggtggtggatgtgtcccacgaggacccagaagtgaagttcaattggtacgtggacggcgtggaagtgcacaacgccaagaccaagcctagagaggaacagtacaactccacctacagagtggtgtccgtgctgaccgtgctgcaccaggattggctgaacggcaaagagtacaagtgcaaggtgtccaacaaggccctggccgctcctatcgaaaagaccatctccaaggccaagggccagcctagggaaccccaggtttacaccttgcctccatctcgggacgagctgaccaagaaccaggtgtccctgtcttgtgccgtgaagggcttctacccctccgatatcgctgtggaatgggagagcaatggccagccagagaacaactacaagacaacccctcctgtgctggactccgacggctcattcttcctggtgtccaagctgacagtggacaagtccagatggcagcagggcaacgtgttctcctgcagcgtgatgcacgaggccctgcacaatcactacacacagaagtctctgtctctgagccccggcaaa

SEQ ID NO: 65 - protein, 455 aa, synthetic construct
QVHLVQSGAEVKKPGASVKISCKASGYILTSYYMQWVRQAPGQGLEWMGIINPSYGGTRYAQKFQGRVTMTRDTSTSTVYMELSSLRSEDTAVYYCARDHLLGPRDYYYYGLDVWGQGTTVTVSSASTKGPSVFPLAPSSKSTSGGTAALGCLVKDYFPEPVTVSWNSGALTSGVHTFPAVLQSSGLYSLSSVVTVPSSSLGTQTYICNVNHKPSNTKVDKKVEPKSCDKTHTCPPCPAPEAAGGPSVFLFPPKPKDTLMISRTPEVTCVVVDVSHEDPEVKFNWYVDGVEVHNAKTKPREEQYNSTYRVVSVLTVLHQDWLNGKEYKCKVSNKALAAPIEKTISKAKGQPREPQVYTLPPSRDELTKNQVSLSCAVKGFYPSDIAVEWESNGQPENNYKTTPPVLDSDGSFFLVSKLTVDKSRWQQGNVFSCSVMHEALHNHYTQKSLSLSPGK

SEQ ID NO: 66 - DNA, 648 bp, synthetic construct
  source 1..648: mol_type = other DNA
  CDS 1..648: protein_id = 67; translation = QSVLTQPPSVSAAPGQKVTISCSGSSSNIGNNYVSWYQQFPGTAPKLLIYDNNKRPSGIPDRFSGSKSGTSATLGITGLQTGDEADYYCGTWDSSLRAHVFGTGTKVTVLGQPKANPTVTLFPPSSEELQANKATLVCLISDFYPGAVTVAWKADGSPVKAGVETTKPSKQSNNKYAASSYLSLTPEQWKSHRSYSCQVTHEGSTVEKTVAPTECS
cagtccgtgctgacccagcctccttctgtttctgctgcccctggccagaaagtgaccatctcttgctccggctcctcctccaacatcggcaacaactacgtgtcctggtatcagcagttccccggcaccgctcctaagctgctgatctacgacaacaacaagcggcccagcggcatccctgacagattctccggatctaagtccggcacctctgctaccctgggcatcacaggattgcagacaggcgacgaggccgactactattgcggcacctgggacagttctctgcgggcccatgtttttggcaccggcaccaaagtgaccgtgctgggacagcctaaggccaatcctaccgtgacactgttccctccatcctccgaggaactgcaggccaacaaggctaccctcgtgtgcctgatctccgacttttaccctggcgctgtgaccgtggcctggaaggctgatggatctcctgtgaaggctggcgtggaaaccaccaagccttccaagcagtccaacaacaaatacgccgcctcctcctacctgtctctgacccctgaacagtggaagtcccaccggtcctactcttgccaagtgacccatgagggctccaccgtggaaaagaccgtggctcctaccgagtgctct

SEQ ID NO: 67 - protein, 216 aa, synthetic construct
QSVLTQPPSVSAAPGQKVTISCSGSSSNIGNNYVSWYQQFPGTAPKLLIYDNNKRPSGIPDRFSGSKSGTSATLGITGLQTGDEADYYCGTWDSSLRAHVFGTGTKVTVLGQPKANPTVTLFPPSSEELQANKATLVCLISDFYPGAVTVAWKADGSPVKAGVETTKPSKQSNNKYAASSYLSLTPEQWKSHRSYSCQVTHEGSTVEKTVAPTECS